European Patent Specification EP 2 951 286 B1, published September 13, 2023. Title: RECOMBINANT MICROORGANISMS COMPRISING NADPH DEPENDENT ENZYMES AND METHODS OF PRODUCTION THEREOF. Applicant: LanzaTech New Zealand Limited. The sequence listing filed with the application follows.

SEQUENCE LISTING (67 sequences)

SEQ ID NO: 1 - DNA, 2226 bp, Unknown
  Clostridium autoethanogenum
atggatattgaggcaccaagagttgccaagtcctgtttaccaggacaatttatcatagtcaaaatggatgataaaggggaaagaatacctcttactatctgtgattatgatgcaggaaaaggaactgttactattgtatttcagacattaggagcttcaactaaaaaaatggctaaatatgaagtgggagaatattttgaagattttgttggaccacttggacattgctcagaacttgtagagatggatcttaaagaacttaagaagaaaaatataatgtttgtagcaggtggtgtaggtactgcaccagtttatccacaggtaaagtggcttcatcagcatggggtagaggcagatgttatagttggatgtaaatcaaaagattatctattatttgaagatgaattaaaaccaatttgtgggaatttatatatagcaacggatgatggaagttatggatataaaggatttgttacggatcttttaaaagagcttattgacaagaaagataaagagtacgattgtgtagttgccatagggcctatgataatgatgaagtttataactcaagttacgaaacaatacggaattaaaacaatagtaagtttaaatactataatggtagatggaactggaatgtgcggagcttgtagggttactgtaggtggagaattaaaatttgcctgtgtagatggtcctgaatttgatggtcatcttgtaaattttgacgaagctatgagaagacaggctatgtataaaactgaagaaggaaagaaacttctgaaagaagaagaaggagacacttttgatagaaaaggctgtgagtgtcacaatgaagataaagctgctaggatgaaaagagtacctataaaggaacaggatcctaaagttagagctactaattttgatgaagtttgcttgggatacactgaagaagaagctgtaaaagaagcttcaagatgcttgaattgtaaaaagcctatgtgtgttactcagtgccctgttacaataactatacctaagtttgttgaacaggtaaaaaatagaaactttgaagaagctgctaaaataatagcagaatcaagtgcacttcctgctgtatgtggaagagtatgtcctcaggaaactcagtgtgaaggaaaatgtgtacttggcaaaaaaggtgatgctgttgctataggtaagctggaaagatttgtagcagattggtcaagaaagaataatatcgatttatctaagactttacctaaaaacggcaaaaaagtagctgttataggaagtggtccttcaggacttacttgtgcaggagatttagcaaagcttggatatgacgttactatatttgaagcacttcatgaagcaggaggagtacttgtatatggtattccagagttcagacttccaaaggatactgtagtaaaacatgaagttgaaaatgtaaagaaattaggagtaaaaatagagacagatgtaataataggaagaactgttactatagatgaactagtagaaaaagaaaaatttgatgctgtatttataggttcaggagcaggactaccaaggtttatgggaatacctggagaaaacttaaatggagtattctctgcaaatgaattcttaacaagaagtaatttaatgaaagcatatagggatgattatgcaactcctataaaagctggtaagaaagtagctgtagtaggaggcggaaacgtagctatggactctgcaaggacagctctaagacttggagcagaagtatacatagtatacagaagatccgaagcagaacttccagcaagagcagaggaagtacaccatgcaaaagaggaaggaataaagttcaatcttttaactaatcctgtagaaatattaggagatgaaaaaggttgggttaatggaatacgctgtattaagatggaacttggagaaccagatgcatctggaagaagaaaaccagttgcaataaagggctcagaatttgatttagatgtagatactgtaattatggcccttggtacttcaccaaatccacttatatcaactacaacaaaaggacttgaaatgaataagcgtaaatgcttaatagcagaagaagagactggacttactacaagagaaggaatatatgcaggtggagatgcagtaacaggtgctgctactgtaatacttgcgatgggtgcaggtaaaaaagctgctaaggctatagatgaatatctgaaaaaataa

SEQ ID NO: 2 - protein, 741 aa, Unknown
  Clostridium autoethanogenum
MDIEAPRVAKSCLPGQFIIVKMDDKGERIPLTICDYDAGKGTVTIVFQTLGASTKKMAKYEVGEYFEDFVGPLGHCSELVEMDLKELKKKNIMFVAGGVGTAPVYPQVKWLHQHGVEADVIVGCKSKDYLLFEDELKPICGNLYIATDDGSYGYKGFVTDLLKELIDKKDKEYDCVVAIGPMIMMKFITQVTKQYGIKTIVSLNTIMVDGTGMCGACRVTVGGELKFACVDGPEFDGHLVNFDEAMRRQAMYKTEEGKKLLKEEEGDTFDRKGCECHNEDKAARMKRVPIKEQDPKVRATNFDEVCLGYTEEEAVKEASRCLNCKKPMCVTQCPVTITIPKFVEQVKNRNFEEAAKIIAESSALPAVCGRVCPQETQCEGKCVLGKKGDAVAIGKLERFVADWSRKNNIDLSKTLPKNGKKVAVIGSGPSGLTCAGDLAKLGYDVTIFEALHEAGGVLVYGIPEFRLPKDTVVKHEVENVKKLGVKIETDVIIGRTVTIDELVEKEKFDAVFIGSGAGLPRFMGIPGENLNGVFSANEFLTRSNLMKAYRDDYATPIKAGKKVAVVGGGNVAMDSARTALRLGAEVYIVYRRSEAELPARAEEVHHAKEEGIKFNLLTNPVEILGDEKGWVNGIRCIKMELGEPDASGRRKPVAIKGSEFDLDVDTVIMALGTSPNPLISTTTKGLEMNKRKCLIAEEETGLTTREGIYAGGDAVTGAATVILAMGAGKKAAKAIDEYLKK

SEQ ID NO: 3 - DNA, 2163 bp, Unknown
  Clostridium ragsdalei
atggatgataaaggggaaagaatacctcttactatctgtgattatgatgcagaaaaaggaactgttactattgtatttcagacattaggagcttcaactaaaaaaatggctaaatatgaagtgggagagtattttgaagattttgttggaccacttggacattgctcagaacttgtagagatggatcttaaagaacttaagaagaaaaatataatgtttgtagcagggggtgtaggtactgcaccagtttatccacaggtaaaatggcttcatgaacatggagttgctgcagatgttatagttggatgtaaatcaaaagatcttttattatttgaagatgaattgaaaccaatttgtggaaatttatatatagcaacggatgatgggagttatggatataagggctttgttacgaatcttttgaaagaacttattgacaagaaagataaagaatatgattgtgtaattgccataggacctatgataatgatgaagtttataactcaagttacgaaaccatatggaattaaaacaatagtaagtttaaatactataatggtagatggaactggaatgtgcggagcttgtagggttactgtaggtggagaattaaaatttgcctgtgtagatggtcctgaatttgatggtcatcttgtaaattttgatgaagctatgagaagacaagctatgtacaagactgaagaaggaaagaaacttctgcaagaagaagaaggggacactggaagtagagaaggtaaaaagtgtagagcagaagaaaaacttgaaagaatgaaaagagtacctataaaggaacaggatcctaaagttagagctactaattttgatgaagtttgcttgggatacactgaagaagaagctgtaaaagaagcttcaagatgcttgaattgtaaaaagcctatgtgtgttactcagtgccctgttacaataactatacctaagtttgttgaacaggtaaaaaatagaaactttgaagaagctgctaaaataatagcagaatcaagtgcacttcctgctgtatgtggaagagtatgtcctcaggaaactcagtgtgaaggaaaatgtgtacttggcaaaaaaggtgatgctgttgctataggtaagctggaaagatttgtagcagattggtcaagaaagaataatatcgatttatctaagactttacctaaaaacggcaaaaaagtagctgttataggaagtggtccttcaggacttacttgtgcaggagatttagcaaagcttggatatgacgttactatatttgaagcacttcatgaagcaggaggagtacttgtatatggtattccagagttcagacttccaaaggatactgtagtaaaacatgaagttgaaaatgtaaagaaattaggagtaaaaatagagacagatgtaataataggaagaactgttactatagatgaactagtagaaaaagaaaaatttgatgctgtatttataggttcaggagcaggactaccaaggtttatgggaatacctggagaaaacttaaatggagtattctctgcaaatgaattcttaacaagaagtaatttaatgaaagcatatagggatgattatgcaactcctataaaagctggtaagaaagtagctgtagtaggaggcggaaacgtagctatggactctgcaaggacagctctaagacttggagcagaagtatacatagtatacagaagatccgaagcagaacttccagcaagagcagaggaagtacaccatgcaaaagaggaaggaataaagttcaatcttttaactaatcctgtagaaatattaggagatgaaaaaggttgggttaatggaatacgctgtattaagatggaacttggagaaccagatgcatctggaagaagaaaaccagttgcaataaagggatcagaatttgatttagatgtagatactgtaattatggcccttggtacttcaccaaatccacttatatcaactacaacaaaaggacttgaaatgaataagcgtaaatgcttaatagcagaagaagagactggactcactacaagagaaggaatatatgcaggtggagatgcagtaacaggtgctgctactgtaatacttgcaatgggtgcaggtaaaaaagctgctaaggctatagatgaatatctgaaaaaataa

SEQ ID NO: 4 - protein, 720 aa, Unknown
  Clostridium ragsdalei
MDDKGERIPLTICDYDAEKGTVTIVFQTLGASTKKMAKYEVGEYFEDFVGPLGHCSELVEMDLKELKKKNIMFVAGGVGTAPVYPQVKWLHEHGVAADVIVGCKSKDLLLFEDELKPICGNLYIATDDGSYGYKGFVTNLLKELIDKKDKEYDCVIAIGPMIMMKFITQVTKPYGIKTIVSLNTIMVDGTGMCGACRVTVGGELKFACVDGPEFDGHLVNFDEAMRRQAMYKTEEGKKLLQEEEGDTGSREGKKCRAEEKLERMKRVPIKEQDPKVRATNFDEVCLGYTEEEAVKEASRCLNCKKPMCVTQCPVTITIPKFVEQVKNRNFEEAAKIIAESSALPAVCGRVCPQETQCEGKCVLGKKGDAVAIGKLERFVADWSRKNNIDLSKTLPKNGKKVAVIGSGPSGLTCAGDLAKLGYDVTIFEALHEAGGVLVYGIPEFRLPKDTVVKHEVENVKKLGVKIETDVIIGRTVTIDELVEKEKFDAVFIGSGAGLPRFMGIPGENLNGVFSANEFLTRSNLMKAYRDDYATPIKAGKKVAVVGGGNVAMDSARTALRLGAEVYIVYRRSEAELPARAEEVHHAKEEGIKFNLLTNPVEILGDEKGWVNGIRCIKMELGEPDASGRRKPVAIKGSEFDLDVDTVIMALGTSPNPLISTTTKGLEMNKRKCLIAEEETGLTTREGIYAGGDAVTGAATVILAMGAGKKAAKAIDEYLKK

SEQ ID NO: 5 - DNA, 882 bp, Unknown
  Clostridium autoethanogenum
atgaatgctcgaagcaaggttatatgtcctttaatcgtagataaggaacgcagttcaaaggcttttactagtgaagctatagatttaattgaaaggagaaagacgaaaaaattaaatgctatatggcttgaagtaacaggatgttcaggaaatatcatttcttttttaaatagtgaaaatcctggactcgattatattttggaaaaactcattaatttaaaatacaacaatactctaatgacttcagaaggggagtatgcctttaaacaattcttagatacattgaatactgaatttatactattagtagatggagcagtatctactgcccagaacggtttttataatattgttgccaattatgaaggaaaccctgttactgcacttgaagctgtaaaaatggcaggagaaaaagcaaagcatgttctctgtgtaggaacttgtgcatcctatggtggaatttctgccgccaggccaaacccttcagaaagcaaaagtgttaaagaaatactaaatcgtgaagtcataagacttccaggctgtccatgccacccggattgggtagttggaactttagcacacttggttgcttttggaaaaccacaattggataaagaaggaagacctcttcttttttatggaattaccattcatgatagttgtacaagaagaggattttttgataacagaatttttgcaaaaaaatttggagaaaatggatgcatgtttaaacttggatgcagggggcctgtaactaaaacagattgtcctaggagaaagtggaatgggtacgtgaactggcctgttgaagacaataccaactgtataggatgtgcaaattctagatttccagatggtatggaaccatttgtaaggtattag

SEQ ID NO: 6 - protein, 293 aa, Unknown
  Clostridium autoethanogenum
MNARSKVICPLIVDKERSSKAFTSEAIDLIERRKTKKLNAIWLEVTGCSGNIISFLNSENPGLDYILEKLINLKYNNTLMTSEGEYAFKQFLDTLNTEFILLVDGAVSTAQNGFYNIVANYEGNPVTALEAVKMAGEKAKHVLCVGTCASYGGISAARPNPSESKSVKEILNREVIRLPGCPCHPDWVVGTLAHLVAFGKPQLDKEGRPLLFYGITIHDSCTRRGFFDNRIFAKKFGENGCMFKLGCRGPVTKTDCPRRKWNGYVNWPVEDNTNCIGCANSRFPDGMEPFVRY

SEQ ID NO: 7 - DNA, 1386 bp, Unknown
  Clostridium autoethanogenum
atgaaaaagaaaattacaattgatccaattacgagaataagcggttttttggaaactaaagtgcaagtagaaaaaaatattatagtagatgctgaaactagtggattgctttttagaggatttgaaaaaatgttaaagaacagagagccgctggatgcagtatattttacagaaagaatttgtggaatatgttcaacagctcatgccgtggcggctgctacagctcttgaagatgctttgaagataaaaattagtgtaaatgattcgtatatgcgtaatttaatacatggttttgaatttatacaaaatcatataagacatttttataatttgaccataccaagttatgtgaagatgcccgatataaatcctctttcttcaaatcaatatgaagattatagattgccttataacctaaataaaaagataagtgaagattatattgaaagtattaaatacagcaggttagcccatgaagggttggctatccttggaggaaaagccccccataatcatggaatttttgttggaggagttaccataaatatagatccatataaactcacaaaagttaaatctattatttctcaaattaataaatttgtaagtagtgttatgttagaggacatgaacataatttcaaaatactatgctgattattttaaaatgggaggagcttatggaaactttatgacttatggaatttttgacaagtatgctgatcctgagataagttatgtaggaccttctgtattaataaatggacgaaagtataatttcaatagtaataaaattacggaaaacatactccacacctggtatacaagcgatgatgaaacgataaatttatctaaagaaacaggttacagctttataaaatcgccaacctataatggatattctatggaagtaggacctctagcaagattgatactttcaggtgagtatactggtggaagttcatgtatggacagaaatgttgccagagtacttgaaacaaaaaagattttagaaattatgcaaggacttgcagatagaattaagcttattccagcagaacaaagaatatatcaaataccagataaagcatttggtgcaggattaattgacacaactagaggatccttgggacactggataagtatagaagataaatttataaagcattacaatattataactcctacagtgtggaatatggggccaagaaatcaatcaggtgcgcttggaattggagaaaaatctttagttggaacgaaaataaaagatataaagcagcctatagaagttgggagaattatgagatcttttgatccttgtgtttcctgtgcaacgcatcttgtaagtgataaatatgaaccagtggatgtacaggttatagtatga

SEQ ID NO: 8 - protein, 461 aa, Unknown
  Clostridium autoethanogenum
MKKKITIDPITRISGFLETKVQVEKNIIVDAETSGLLFRGFEKMLKNREPLDAVYFTERICGICSTAHAVAAATALEDALKIKISVNDSYMRNLIHGFEFIQNHIRHFYNLTIPSYVKMPDINPLSSNQYEDYRLPYNLNKKISEDYIESIKYSRLAHEGLAILGGKAPHNHGIFVGGVTINIDPYKLTKVKSIISQINKFVSSVMLEDMNIISKYYADYFKMGGAYGNFMTYGIFDKYADPEISYVGPSVLINGRKYNFNSNKITENILHTWYTSDDETINLSKETGYSFIKSPTYNGYSMEVGPLARLILSGEYTGGSSCMDRNVARVLETKKILEIMQGLADRIKLIPAEQRIYQIPDKAFGAGLIDTTRGSLGHWISIEDKFIKHYNIITPTVWNMGPRNQSGALGIGEKSLVGTKIKDIKQPIEVGRIMRSFDPCVSCATHLVSDKYEPVDVQVIV

SEQ ID NO: 9 - DNA, 1398 bp, Unknown
  Clostridium autoethanogenum
atgttaaatatgccaactagtacttctatgataaatatagatgaagaattatgtacaggctgcagacgatgtgcggatgtctgccctgtagatgctatagaaggtgaacagggtaaacctcagaagataaatactgaaaagtgtgttatgtgcggacaatgcattcaagtttgtaaaggctatcaatctgtatacgacgatgttcctactccagttagcaaaaggttatttgatagaggattgttaaaggaagtagatgaaccattatttgcagcatataataaaggtcaggtaaagagtgttaaagaaattttacaaaacaaagatgtatttaaaattgtgcaatgtgcacctgctgtaagagttgctataggagaggattttggaatgcctcttggaactttaagtgaaggaaaaatggcagctgcactcagaaaattaggatttgacaaagtatatgatacaaactttggtgcagatcttactataatggaagaaggtagtgagttactaaaaagagtagctgaaggcggagttttgccaatgtttacttcttgttgtccagcatgggtaaaatatgcagaacaaacatatccagaacttttacctcatctttcaagttgtaagtctccaaatcagatggctggagctatatttaaaacttatggagcagagataaataaggttaatccggctaaaatttataatgtatctgttatgccatgtacatgcaaggaatttgaaagtgaaagagaagaaatgcatgacagtggacacagggatgtagatgcagttataactacaagggaattagcacaactgttcaaagatgctgatatagattttaatactattgaagaagaacagtttgatactcctcttggtatgtataccggtgcaggaactatatttggtgctacaggtggagttatggaagcagcacttagaactggatatgaactttatactaaaaaaactattccaagtatagatcttactatggtaagaggtggagaaggttttagaactgctgaagtagatttaggggatattagactaaaagtaggagtagtttccggcttaaaaaatgtaaaagacgttatggaatcagtaaaggcaggcaaatgtgatttgcactttatagaggttatgacctgtcctcaaggatgtataagtggtggaggacaacctaaagttatacttgattcagataaagaggaagcttataataataggaaaaagggactatataatcatgacgctaatcttacttatagaaaatcacatgaaaatccagaaataaagaaaatatatgatgagttcttagacaaaccattaggagctaagtctcatgaattattgcacactaaatatatctcaagaaaaaaggagagttaa

SEQ ID NO: 10 - protein, 465 aa, Unknown
  Clostridium autoethanogenum
MLNMPTSTSMINIDEELCTGCRRCADVCPVDAIEGEQGKPQKINTEKCVMCGQCIQVCKGYQSVYDDVPTPVSKRLFDRGLLKEVDEPLFAAYNKGQVKSVKEILQNKDVFKIVQCAPAVRVAIGEDFGMPLGTLSEGKMAAALRKLGFDKVYDTNFGADLTIMEEGSELLKRVAEGGVLPMFTSCCPAWVKYAEQTYPELLPHLSSCKSPNQMAGAIFKTYGAEINKVNPAKIYNVSVMPCTCKEFESEREEMHDSGHRDVDAVITTRELAQLFKDADIDFNTIEEEQFDTPLGMYTGAGTIFGATGGVMEAALRTGYELYTKKTIPSIDLTMVRGGEGFRTAEVDLGDIRLKVGVVSGLKNVKDVMESVKAGKCDLHFIEVMTCPQGCISGGGQPKVILDSDKEEAYNNRKKGLYNHDANLTYRKSHENPEIKKIYDEFLDKPLGAKSHELLHTKYISRKKES

SEQ ID NO: 11 - DNA, 1680 bp, Unknown
  Clostridium autoethanogenum
atgagtggacaatttatgattatagataatattcctgtagagataaatggtgaaaaaaatattcttgaactaattagaaaagctggcattgatttacctacattttgctatcattcggagctttcagtttatggtgcatgccgtatgtgcatggttgaagataaacgcggccgtatgcaagctgcatgttctactcctcctcaagctggtatagaaatatatacaaatactccaagacttagaaaatacagaaaaaacattcttgagttgttactcgcaaatcattgcagagattgtacaacttgtgaaaaaaatgagcattgcaaactacaagatttagcaaagcgttttaaaataaagaaagtaagatttaaaaatacttctataaataaaaaaattgataattcatcagtatgcattgtaagaaataggagtaaatgtatcttatgcggtgactgtgtaagagtgtgtgaagaagtacaaaatgttggagctattgattttgttaaaagaggttctaatatgactgtaactactgcatttgatgaacctatagcaaattcgaattgtgttggatgtggtcaatgtgcggcagtatgccctactggtgctattgtagtaaaggatgatacagctgaattatgggaagcacttagtgataagaatacaaaggttgtagctcaaattgcgcccgctgtaagagttggtcttaatgaggaattaggtgaggaaaacggcgaaaacgaaatgggtaaaatagtagctgcacttagaagaatgggatttgatgaagtttttgatacttcaacggcagcagatcttacagttttggaagaaacagcagaatttacttcaagacttgaaaaaaatgaaagtttaccattgtttacatcctgttgttctgcatgggtaaattatgtagagaatacacatccagagttaatgaaatatgtttctacttgcaaatcacctatggaaatgtttgcttctgtacttaaggagtactataaaaatagtgataaaaaaattgtagttgtagcagttatgccttgtacagctaaaaaatatgaagcaaaacgagaagaattttcaaaaaatggtgtacctgatgtagattatgtaataactacacaggagcttataagtatgataagacaagcaggaattgtatttcctgaattagagcctgaagcagttgatatgccatttgatcttagcagtggagctggagttatatttggagtaacaggtggtgttacagaggctgttatacgtaaagttttagctgataaatcaaatgctgcattacgtgcaattgtgtttaatggtgttaggggcatggaaggtactaaagaagctagcattactgttggtgatcgtgaaataaaaatagcaatagtaagcggtcttagaaatgcagaaaatcttatacagaaaatacaatctggtgaatcaaaatatgatttcgttgaagttatggcatgtccaggtggatgcatttctggtggtggacaaccatttgaaaaacttgaaggaaagctaaaacgtagtgctggaatatatcaatcagataaaatgagcactataaaacgtacagctgacaatccgcttatgaaatcactgtattcaggattgttaaaaggtaaaaaccacgaactattacatgtaaaccgcaaatag

SEQ ID NO: 12 - protein, 559 aa, Unknown
  Clostridium autoethanogenum
MSGQFMIIDNIPVEINGEKNILELIRKAGIDLPTFCYHSELSVYGACRMCMVEDKRGRMQAACSTPPQAGIEIYTNTPRLRKYRKNILELLLANHCRDCTTCEKNEHCKLQDLAKRFKIKKVRFKNTSINKKIDNSSVCIVRNRSKCILCGDCVRVCEEVQNVGAIDFVKRGSNMTVTTAFDEPIANSNCVGCGQCAAVCPTGAIVVKDDTAELWEALSDKNTKVVAQIAPAVRVGLNEELGEENGENEMGKIVAALRRMGFDEVFDTSTAADLTVLEETAEFTSRLEKNESLPLFTSCCSAWVNYVENTHPELMKYVSTCKSPMEMFASVLKEYYKNSDKKIVVVAVMPCTAKKYEAKREEFSKNGVPDVDYVITTQELISMIRQAGIVFPELEPEAVDMPFDLSSGAGVIFGVTGGVTEAVIRKVLADKSNAALRAIVFNGVRGMEGTKEASITVGDREIKIAIVSGLRNAENLIQKIQSGESKYDFVEVMACPGGCISGGGQPFEKLEGKLKRSAGIYQSDKMSTIKRTADNPLMKSLYSGLLKGKNHELLHVNRK

SEQ ID NO: 13 - DNA, 1917 bp, Unknown
  Clostridium autoethanogenum
gtgaataaaagtcctgtaactgttttaaaagaaaaatgtacaggttgtaataagtgtataagaacttgtcctattcttggtgcaaatgttacagcaactgaaaatggtgtaagtaaggtttacatagatgaggaaagatgtattggatgcggtgaatgtgtaaaggtttgcgaacatggggctagagactttaacgatagtacacaagacttttttaaggatttgaaaaaaggcaaaaaaataacagtaatagctgcaccatctattatagttaatattaaaaattacaagaaattttttggatatcttaaatctttgggagtatctataatttatgatgtttctttcggtgcagatattactacctgggcttatctaaaagcaatgaaggagaaaaatatttcttctttaatatcacagccctgtcctatcgtggttaattatattgaaaaatataagcctgaattaatagaatatttagcgcctatacacagtcctatgatgtgtactgctgtttatctgaaaaaatataagcatatatgtgaagatatagcttttctgtcaccttgtattggcaagctaattgaaatcaatgataagaatacagatgggtatgtgaaatataatgtaacgtacaaaaagattttagattatttgagagataataatgtgaatttgaacaattacgatgaagttgaatttgataatgttcctgcttctttgggggttgtttatagtttaccaggtggattaaaagcaaatgtaaaagctagaactgaagaactacatgttcttcagatagaaggacacaaagaggcaattgagtacttgaataagtattctgatagagttaaagctaataaacttatacctagtttacttgatattttaaattgcaaaaatggatgtaatataggtacagcttccttagacaatttaacggaatatgatattcaatataggtttcatgatataaaggtggaaaagttaagagaaaaaactggcttgtttaagaaaaaaatcaaatcaatagacgagtactttgataaaaatcttaatttaaacgattttgtaagaaagtatactgcacagaaggttaaaaaaataattgaacctacccaaaaagattatgacaacatatttgatgagatgatgaaaactacaacattgggaaaagaattcaattgttccgcttgtggatacagcacttgcaaagaaatggtaaagatgatttttaacggcataaattctaaggaaaattgtatttattatgtgaagaaaaaaatcaatatggaatatagcgaactggaagaaaaaaatgaagaggtcaaagagtctataaacaaaataactgtactagctgaggaaagacaacgaaaatcagatgaaataattaaatttgcaaatactctattggcagctataaatgaagtaagtaaagggaatgaggaaagcgcatctgcaattcaagatatagtagaagaattaaagtcaataatggatatatcaagtaagttaaaggaaaacattcatcagataaatgaaaagttagacaaattcacggattcatcagatagtattgtggctatttcagagcagactaatttactttcgctaaatgccgcaatagaagcagcacgggcaaatgaacatggaaaaggttttgcagtagtagcagatgaagtaaagaagctagcagagcaatctaaaactaccgcacaatctactaaaaacgaagaaaatgaaatgatgcaatctattttaaaggttattgaagtatctgatttacttcagaacaaaatggataatataaataacgatatattaactatatcggaaactatccaagagataagtgctaagagtcaggagatagtttctagctctgaaaagttaataaacagtgagtcacattaa

SEQ ID NO: 14 - protein, 638 aa, C. autoethanogenum
MNKSPVTVLKEKCTGCNKCIRTCPILGANVTATENGVSKVYIDEERCIGCGECVKVCEHGARDFNDSTQDFFKDLKKGKKITVIAAPSIIVNIKNYKKFFGYLKSLGVSIIYDVSFGADITTWAYLKAMKEKNISSLISQPCPIVVNYIEKYKPELIEYLAPIHSPMMCTAVYLKKYKHICEDIAFLSPCIGKLIEINDKNTDGYVKYNVTYKKILDYLRDNNVNLNNYDEVEFDNVPASLGVVYSLPGGLKANVKARTEELHVLQIEGHKEAIEYLNKYSDRVKANKLIPSLLDILNCKNGCNIGTASLDNLTEYDIQYRFHDIKVEKLREKTGLFKKKIKSIDEYFDKNLNLNDFVRKYTAQKVKKIIEPTQKDYDNIFDEMMKTTTLGKEFNCSACGYSTCKEMVKMIFNGINSKENCIYYVKKKINMEYSELEEKNEEVKESINKITVLAEERQRKSDEIIKFANTLLAAINEVSKGNEESASAIQDIVEELKSIMDISSKLKENIHQINEKLDKFTDSSDSIVAISEQTNLLSLNAAIEAARANEHGKGFAVVADEVKKLAEQSKTTAQSTKNEENEMMQSILKVIEVSDLLQNKMDNINNDILTISETIQEISAKSQEIVSSSEKLINSESH

SEQ ID NO: 15 - DNA, 1347 bp, Unknown
  Clostridium autoethanogenum
ttgagagatgattataggaatctatttaaattcataataaaggcatattatagtggaaattttgaagaagaagtgatgtcatttttattagagtctaaaatggataaacaggaattgtgtaagattatatctacgttgtgcggcactaatatagattatagttccaattttatagaaaatttgaaaaaagcaataaagtcttataaacaagaaggtaaagtagtcaataaagttagagactgttccatggaatgtgtggatgaaaaaggtgagatactttgtcaaaaaacatgtccttttgatgcaatttttatagacaataagaaaaattgtgcttacatagataaagaaaaatgtaccgattgtggtttttgtgtagatgtttgtcctactgggggaataatggataaagttcagttcattcctcttgctgatattttaaaaagcaaatctccagttgtggctatagtggctcctgccataataggacagtttggcgaagatgttactatggatcaacttaggactgcttttaaaaaactgggatttactgatatgattgaagtggcattttttgcagatatgcttactttaaaggagtctattgaatttgacaatcatgtaaaagatgaaaaagattttatgataacctcctgctgctgccctatgtgggtagctatggtaaaaaaggtatacagtaatttggttaaacacgtatccccctctgtatctccaatggttgcaggaggaagagtacttaaaaagttaaacccttactgcaaggtagtgtttataggaccatgtattgctaaaaaatctgaggcaaaggaagaagacataaaaggagcaatagatttcgtacttacttttgaagaattaagagatatatttgatgcttttcatatagttccatctaaacttgaaggagatttttcctctaaatatgcgtctaggggtggaagattatatgctcgtacagggggagtttctattgcagtaagcgaagctgtggaaagaattttccctgaaaagcataaactatttagtgcaattcaggcaaatggcattagagaatgtagagaaatgcttaccaaggtgcaaaatggagaaataaaagctaattttattgaaggaatgggctgcattggcggatgtgtaggtggtcccaaagcaattgtacttaaggatgaaggtagggatcgagtaaataaatttgcacaagattctgaaataaaagttgctgtagatagtgaatgcatgcatggagtattacatgctttggatatacattctatagatgattttaaggatgagaaaaaaatagaactgttagaacgagaattttaa

SEQ ID NO: 16 - protein, 448 aa, Unknown
  Clostridium autoethanogenum
MRDDYRNLFKFIIKAYYSGNFEEEVMSFLLESKMDKQELCKIISTLCGTNIDYSSNFIENLKKAIKSYKQEGKVVNKVRDCSMECVDEKGEILCQKTCPFDAIFIDNKKNCAYIDKEKCTDCGFCVDVCPTGGIMDKVQFIPLADILKSKSPVVAIVAPAIIGQFGEDVTMDQLRTAFKKLGFTDMIEVAFFADMLTLKESIEFDNHVKDEKDFMITSCCCPMWVAMVKKVYSNLVKHVSPSVSPMVAGGRVLKKLNPYCKVVFIGPCIAKKSEAKEEDIKGAIDFVLTFEELRDIFDAFHIVPSKLEGDFSSKYASRGGRLYARTGGVSIAVSEAVERIFPEKHKLFSAIQANGIRECREMLTKVQNGEIKANFIEGMGCIGGCVGGPKAIVLKDEGRDRVNKFAQDSEIKVAVDSECMHGVLHALDIHSIDDFKDEKKIELLEREF

SEQ ID NO: 17 - DNA, 1374 bp, Unknown
  Clostridium autoethanogenum
ttgacagttaaaagtgaaggtattgtcaaaattgataaagagttgtgtacaggatgtagacgatgtgcagatatttgtcctgtagatgctatagaaggtgagaagggacaacctcaaacaattaatactgaacgctgtgttttgtgtggtcagtgtgtacaaatttgcagtgcttatgcatctgcatttgatgaagatattactcctcataaggaaaagataaaagagcgtaatatgcttccatctgttaaagagcccttatttgcatcctactatagaggagatgctccagcagtaaaagaggccttagcaaattctaaactttttactatggttcaatgcgcaccagcagtacgtgtggctattgccgaagaatttggtatgccacttggaagtttaacaccagggaaaatggcagctgcgctaagagagttaggttttgatcgaatttatgatactaattttgctgctgatctaactattatggaggaaggcagtgaacttattaaaagggttactgaaggtggagtactgccaatgttcacttcatgttgtcctgcttgggtaaaatttattgagcaggattatccggaacttattccacatctgtcttcttgtaaatctccgcagcaaatggaaggtgctctgcttaaaacatatggtgcacaggttgatggtgtagatgctggcaagatttatagtgtttcagttatgccttgtatttgcaaaaaatttgaatgtgaacgtcctgaaatgaaagacagtggatatcaggatgtagatgctgtaattaccacacgggaacttgcacaattaatcaaggatgatggcattgattttaatggtttacctgaaaaagaatttgacaagccacttggaacttattctggtgcaggcactattttctgtgctactggtggtgttatggaagctgccctgcgtacggcatataaattgattactaaagaagagattccagatgtcgatctcaaattcataagaggaggcgaaggcgcaagaagttcagaaattaaagtaggagatttaacactaaaagtagcagtagttgctggtctgaaaaatgttgtaccagttttggaagcaattaaaactgggaaagcagatttccatttcattgaagtgatgacctgtccagttggatgtgttagcgggggcggacaacctaaggtattgatacctgatgaaaaagctgattcgtatactaatcgtacatgcagtacgtatgtacatgatgaaaatatggaatatagaaaatcacatgataatcctgaaatacagaaaatttataaagaattcttggtagaagataatattcatcatttgcttcatactacgtatacgccaaggaggtaa

SEQ ID NO: 18 - protein, 457 aa, Unknown
  Clostridium autoethanogenum
MTVKSEGIVKIDKELCTGCRRCADICPVDAIEGEKGQPQTINTERCVLCGQCVQICSAYASAFDEDITPHKEKIKERNMLPSVKEPLFASYYRGDAPAVKEALANSKLFTMVQCAPAVRVAIAEEFGMPLGSLTPGKMAAALRELGFDRIYDTNFAADLTIMEEGSELIKRVTEGGVLPMFTSCCPAWVKFIEQDYPELIPHLSSCKSPQQMEGALLKTYGAQVDGVDAGKIYSVSVMPCICKKFECERPEMKDSGYQDVDAVITTRELAQLIKDDGIDFNGLPEKEFDKPLGTYSGAGTIFCATGGVMEAALRTAYKLITKEEIPDVDLKFIRGGEGARSSEIKVGDLTLKVAVVAGLKNVVPVLEAIKTGKADFHFIEVMTCPVGCVSGGGQPKVLIPDEKADSYTNRTCSTYVHDENMEYRKSHDNPEIQKIYKEFLVEDNIHHLLHTTYTPRR

SEQ ID NO: 19 - DNA, 1737 bp, Unknown
  Clostridium autoethanogenum
atggtaaatttaactataaacgatataaaggtttctgtcccagaaggcactacaattttaaacgctgcaaaaaaagtaaacataaatatacctactctctgctatcttgatcttcacgatataaaaatggtaaatagaacttcctcctgcagagtttgtcttgttgaaattgaaggaagacgaaatcttgcaccttcatgttctacagaagctttcgagggtatgatagttagaacaaacagtgccagagctataaaagcaaggcgtaccatggtagaacttttattatcagatcatcctaccgactgccttgtatgtgaaaagaatactcaatgccaacttcaattaattgctgctgaattaggtataaggaaaataagatataaaggtgctatgtctaattataagaaggattcctccagcggtgctctatatagaaatctggataagtgcataatgtgcagacgatgcgaaaccatgtgcaatgaagttcaaacctgtcaggtttactctgcagtagatagaggcttcgaaactgtagtatcccctgcatttggtcgtcctatggttgacacgcaatgcacattttgcggtcaatgtgtatcagtatgtccaaccgctgcattaactcaagttagtaatgtagctaaggtatgggaagtactaactgatcctgataaatatgtagtagttcaaactgcccctgctataagagttactttaggtgaaaaattcggtatggaacctggaactattgtaactggcaaaatggttgcagccttaagaagattgggttttgataaggtatgtgatacagactttgcagcagatgtaactattttagaagaagctcatgaatttatagatagacttcaaaatggtggaagacttccaatactcacaagctgctgtcccagctgggttaaatttatagaacatcaatttcctgatcttttagatataccttcaacttgtaaatctccacacataatgtttggtactttagctaaaacatatatggcagaaaaattaaatattgatccatctaaaattgtagtagtttcagttatgccctgtattgcaaaaaaatatgaaataagcagaaaagagcttcaatatgaaggtcataaaaatgttgatcttgtggttaccacaagagagcttgcagatatgataatggaagcaggaatagattttaacaaacttcctgatgaagattttgataatccacttggagaatccacaggtgcctctgtaatatttggaactaccggcggcgtaattgaagcagctcttagaactgcttatgaatggattactggagagactttaaaagaagtagaatttcatagtgtaagaggtcttgacggacttaaagaagccagtataaatattggtggtaaaaaaataaacatcggtgtagcacacggtcttggcaacgcaagaaaacttcttgaggaaatagaatctggtgaatcaaaatatcatgctatagaaataatggcctgtcctggaggatgtattgacggaggaggtcagccatatcactttggagatttagatatcgtaaagaaaagaatggaagctttatatagagaagatagaaacaaacctctcagaaaatctcatgaaaatcctgaagttcaagctctatataaagaatttattggtgatgtaggtggaaaaaaagctcatgatctccttcacacccattatataaaaaggcaaaaattataa

SEQ ID NO: 20 - protein, 578 aa, Unknown
  Clostridium autoethanogenum
MVNLTINDIKVSVPEGTTILNAAKKVNINIPTLCYLDLHDIKMVNRTSSCRVCLVEIEGRRNLAPSCSTEAFEGMIVRTNSARAIKARRTMVELLLSDHPTDCLVCEKNTQCQLQLIAAELGIRKIRYKGAMSNYKKDSSSGALYRNLDKCIMCRRCETMCNEVQTCQVYSAVDRGFETVVSPAFGRPMVDTQCTFCGQCVSVCPTAALTQVSNVAKVWEVLTDPDKYVVVQTAPAIRVTLGEKFGMEPGTIVTGKMVAALRRLGFDKVCDTDFAADVTILEEAHEFIDRLQNGGRLPILTSCCPSWVKFIEHQFPDLLDIPSTCKSPHIMFGTLAKTYMAEKLNIDPSKIVVVSVMPCIAKKYEISRKELQYEGHKNVDLVVTTRELADMIMEAGIDFNKLPDEDFDNPLGESTGASVIFGTTGGVIEAALRTAYEWITGETLKEVEFHSVRGLDGLKEASINIGGKKINIGVAHGLGNARKLLEEIESGESKYHAIEIMACPGGCIDGGGQPYHFGDLDIVKKRMEALYREDRNKPLRKSHENPEVQALYKEFIGDVGGKKAHDLLHTHYIKRQKL

SEQ ID NO: 21 - DNA, 882 bp, Unknown
  Clostridium ragsdalei
atgaatgttcgaaacaagggtatatgtcctttaatcgtagataaggaacgcagttcaaaggcttttactagtgaagctatagatttaattaaaaggggaaagacgaaaaaattaaatgctatatggcttgaagtaacaggatgttcaggaaatattatttcttttttaaatagtgaaaatcctggactcgattatattttagaaaaactcattaatttaaaatacaacaatactctaatgacttcagaaggtgagtatgcttttaaacaattcttagatacattggatactgaatttatactactagtagatggagcggtatctactgctcaaaatggtttttataatattgttgccaattatgaaggaaaacctgttactgcacttgaagctgtaaaaatggcaggagaaaaagcaaagtatgttctctgtgtaggaacttgtgcatcctatggtggaatttctgccgccaggccaaacccatcagaaagcaaaagtgttaaagaaatactaaatcgtgaagtcataagacttccaggctgtccatgccatccggattgggtagttggaactttagcacatttagttgcttttggcaaaccgcaattggatgaagatggaagacctcttcttttttatggaattaccattcatgataggtgtacaagaaggggattttttgataacagaatttttgcaaaaaaatttggagaagatggatgtatgtttaaacttggatgcagggggcctgtaactaaaacagattgtcctaggagaaagtggaatggatatgtgaactggcctgttgaagacaataccaactgtataggatgtgcaaattctagatttccagatggtatggaaccatttgtaaggtattag

SEQ ID NO: 22 - protein, 293 aa, Unknown
  Clostridium ragsdalei
MNVRNKGICPLIVDKERSSKAFTSEAIDLIKRGKTKKLNAIWLEVTGCSGNIISFLNSENPGLDYILEKLINLKYNNTLMTSEGEYAFKQFLDTLDTEFILLVDGAVSTAQNGFYNIVANYEGKPVTALEAVKMAGEKAKYVLCVGTCASYGGISAARPNPSESKSVKEILNREVIRLPGCPCHPDWVVGTLAHLVAFGKPQLDEDGRPLLFYGITIHDRCTRRGFFDNRIFAKKFGEDGCMFKLGCRGPVTKTDCPRRKWNGYVNWPVEDNTNCIGCANSRFPDGMEPFVRY

SEQ ID NO: 23 - DNA, 1386 bp, Unknown
  Clostridium ragsdalei
atgaaaaagaaaattaccattgatccaattacgagaataagtggttttttggaaactaaagtgcaagtagaaaaaaatattatagtagatgctgaaactagtggattgctttttagaggatttgaaaaaatgttaaaaaacagacagccgctggatgcagtatattttacagaaagaatttgtgggatatgttcaacagctcatgctgtggcagctgctacagctcttgaagatgctttgaagataaaaattagtgtaaatgattcgtatatgcgtaatttaatacatggttttgaatttatacaaaatcatataagacatttttataatttgactataccaagttatgtgaagatgcccaatataaatcctcttttttcagatcaatatgaagattatagattaccttataacttaaataaaaagataagtgaagattatattgaaagtattaaatacagtaggttagcccatgaaggattggctactcttggaggaaaggctccccataatcacggaatttttgttggaggagttaccataaatatagatccatataaacttacaaaagttaaatctattatttctcaaattaatgaattcgtaagtagtgttatgttagaggacatgaacataatttcaaaatactatgctgattattttaaaatgggaaaagcctatggaaactttatgacttatggaatttttgataagtatgctgatcctgagataagttatgtaggaccttctgtcttaataaatggacaaaagcataactttaatagtaataaaattacagagaatatactttacacctggtacatgaatgatgatgaaacaataaatttatctaaagaaacaggttacagctttataaaatcgccaacttatgatggctattctatggaagtaggacctctagcaagattgatactttcaggtgagtatactggtggaagttcatgtatggacagaaatgttgccagagtacttgaaacaaaaaagattttagaaattatgcaaggacttgcagatagaattaagcttattccagcagaacaaagaatatatgaaatcccagataaagcatttggtgcaggattaattgacacaactagaggatccttgggacactggataagtatagaagataaatttataaagcattacaatattataactcctacagtgtggaacatggggccaagaaatcaatcaggtgcgcttggaattggagaaaaatctttacttggaacgaaaataaaagatataaagcagcctatagaagttgggagaattatgaggtcctttgatccttgtgtttcctgtgcaactcatttgataagtgatgcatatgaaccagtggacgtacaggttatagtatga

SEQ ID NO: 24 - protein, 461 aa, Unknown
  Clostridium ragsdalei
MKKKITIDPITRISGFLETKVQVEKNIIVDAETSGLLFRGFEKMLKNRQPLDAVYFTERICGICSTAHAVAAATALEDALKIKISVNDSYMRNLIHGFEFIQNHIRHFYNLTIPSYVKMPNINPLFSDQYEDYRLPYNLNKKISEDYIESIKYSRLAHEGLATLGGKAPHNHGIFVGGVTINIDPYKLTKVKSIISQINEFVSSVMLEDMNIISKYYADYFKMGKAYGNFMTYGIFDKYADPEISYVGPSVLINGQKHNFNSNKITENILYTWYMNDDETINLSKETGYSFIKSPTYDGYSMEVGPLARLILSGEYTGGSSCMDRNVARVLETKKILEIMQGLADRIKLIPAEQRIYEIPDKAFGAGLIDTTRGSLGHWISIEDKFIKHYNIITPTVWNMGPRNQSGALGIGEKSLLGTKIKDIKQPIEVGRIMRSFDPCVSCATHLISDAYEPVDVQVIV

SEQ ID NO: 25 - DNA, 1398 bp, Unknown
  Clostridium ragsdalei
atgttaaatatgccaactagtacttctatgataaatatagatgaagaattatgtacaggctgcagacgatgtgcggatgtctgccctgtagatgctatagaaggtgaacagggtaaacctcagaagataaatactgaaaagtgtgttatgtgcggacaatgcattcaagtttgtaaaggctatcaatctgtatacgatgatattcctactccagttagcaaaaggttatttgatagaggattgttaaaggaagtagatgaaccattatttgcagcatataataaaggtcaggcaaagagagttaaagaaattttacaaaacaaagatgtatttaaaattgtgcaatgtgcacctgctgtaagagttgctataggagaggattttggaatgcctcttggaactttaagtgaaggaaaaatggcagctgcactcagaaaattaggatttgacaaagtatatgatacaaactttggtgcagatcttactataatggaagaaggtagtgagttactaaaaagagtagctgaaggtggagttttgccaatgtttacttcttgttgtccagcatgggtaaaatatgcagaacaaacatatccagaacttttacctcatctttcaagttgtaagtctccaaatcagatggctggagctatatttaaaacttatggagcagagataaataaggttaatccggctaaaatttataatgtatctgttatgccatgtacatgcaaggaatttgaaagtgaaagagaagaaatgcatgacagtggacacagagatgtagatgcagttataactacaagggaattagcacaactgttcaaagatgctgatatagattttaatactattgaagaagaacagtttgatactcctcttggtatgtatactggtgcaggaactatatttggtgctacaggtggagttatggaagcagcacttagaactggatatgaactttatactaaaaaaactattccaagtatagatcttactatggtaagaggtggagaaggttttagaactgctgaagtagatttaggagatattagactaaaagtaggagtagtttccggcttaaaaaatgtaaaagatgttatggaatcagtaaaggcaggtaaatgtgatttacactttatagaggttatgacttgtcctcaaggatgtataagtggtggaggacaacctaaggttatacttgattcagataaagaagaagcttataataataggaaaaagggactatataatcatgacgctaatcttacttatagaaaatcacatgaaaatccagaaataaagaaaatatatgatgagttcttagacaaaccattaggagctaagtctcatgaattattgcacactaaatatatctcaagaaaaaaggagagttaa

SEQ ID NO: 26 - protein, 465 aa, Unknown
  Clostridium ragsdalei
MLNMPTSTSMINIDEELCTGCRRCADVCPVDAIEGEQGKPQKINTEKCVMCGQCIQVCKGYQSVYDDIPTPVSKRLFDRGLLKEVDEPLFAAYNKGQAKRVKEILQNKDVFKIVQCAPAVRVAIGEDFGMPLGTLSEGKMAAALRKLGFDKVYDTNFGADLTIMEEGSELLKRVAEGGVLPMFTSCCPAWVKYAEQTYPELLPHLSSCKSPNQMAGAIFKTYGAEINKVNPAKIYNVSVMPCTCKEFESEREEMHDSGHRDVDAVITTRELAQLFKDADIDFNTIEEEQFDTPLGMYTGAGTIFGATGGVMEAALRTGYELYTKKTIPSIDLTMVRGGEGFRTAEVDLGDIRLKVGVVSGLKNVKDVMESVKAGKCDLHFIEVMTCPQGCISGGGQPKVILDSDKEEAYNNRKKGLYNHDANLTYRKSHENPEIKKIYDEFLDKPLGAKSHELLHTKYISRKKES

SEQ ID NO: 27 - DNA, 1737 bp, C. ragsdalei
atggtaaatttaactataaacgatataaaggtttctgtcccagaaggcactacaattttaaacgctgcaaaaaaagtaaacataaatatacctactctctgctatcttgatcttcacgatataaaaatggtaaataggacttcctcctgcagagtctgccttgttgaaattgaaggcaggcgaaatcttgcaccttcatgttctacagaagctttcgaaggtatgatagttagaacaaatagtgccagagctataaaagcaaggcgtactatggtagaacttttattatcagatcatcctaccgactgccttgtatgtgaaaagaatactcaatgtcaacttcaattaatcgctgctgaattaggtataagaaaaataagatataaaggtgctatgtctaattacaaaaaggattcatcaagtggtgctatatatagaaatcttgataaatgtataatgtgcagacgatgtgaaaccatgtgcaatgaagttcaaacctgtcaggtttactctgcagtagatagaggcttcgaaactgtagtatcccctgcatttggtcgtcccatggttgacacgcaatgcacattttgcggtcaatgtgtatccgtatgcccaactgctgcattaactcaagttagtaatgtagctaaggtatgggaagtactaactgatcctgataaatatgtagtagttcaaactgcccctgctataagagttactttaggtgaaaaattcggtatggaacctggaactattgtaactggcaaaatggtatctgctcttagaagattgggctttgataaggtatgtgataccgattttgcagcagatgtaactattttagaagaagctcatgaatttatagatagacttcaaaacggcggaagacttccaatactcacaagctgctgtcccagctgggttaaatttatagaacatcaatttcctgatcttttagatataccttcaacttgtaagtctccacacataatgtttggtactttagctaaaacatatatggcagaaaaattaaatattgatccatctaaaattgtaatagtttcagttatgccatgtattgcaaaaaaatatgaagtaagcagaaaagaacttcaatatgaaggtcataaaaatgttgatcttgtagttaccacaagagagcttgcagatatgataatggaagcaggaatagattttaataaacttcctgatgaagactttgataaaccttttggagaatccacaggtgcttctgtaatatttggaactaccggcggtgtaattgaagcagctcttagaactgcttatgaatggattactggagagactttaaaagaagtagaatttcatggtgtaagaggacttgatggacttaaagaagccagtataaatattggtggtaaagaaataaacattggcgtagctcacggtcttggcaacgcaagaaaacttcttgaggaaatagaatctggtgaatcaaaatatcacgctatagaaataatggcatgtcctggaggatgtattgacggaggaggtcagccgtatcattttggagatttagatattgtaaagaaaagaatggacgctttatatagagaagatagaaacaaacctctcagaaaatctcatgagaatcctgaagttcaagctctatataaagaatttattggagatgtaggcggaaaaaaagctcatgatctccttcacactcattatataaaaaggcaaaagttataa

SEQ ID NO: 28 - protein, 578 aa, C. ragsdalei
MVNLTINDIKVSVPEGTTILNAAKKVNINIPTLCYLDLHDIKMVNRTSSCRVCLVEIEGRRNLAPSCSTEAFEGMIVRTNSARAIKARRTMVELLLSDHPTDCLVCEKNTQCQLQLIAAELGIRKIRYKGAMSNYKKDSSSGAIYRNLDKCIMCRRCETMCNEVQTCQVYSAVDRGFETVVSPAFGRPMVDTQCTFCGQCVSVCPTAALTQVSNVAKVWEVLTDPDKYVVVQTAPAIRVTLGEKFGMEPGTIVTGKMVSALRRLGFDKVCDTDFAADVTILEEAHEFIDRLQNGGRLPILTSCCPSWVKFIEHQFPDLLDIPSTCKSPHIMFGTLAKTYMAEKLNIDPSKIVIVSVMPCIAKKYEVSRKELQYEGHKNVDLVVTTRELADMIMEAGIDFNKLPDEDFDKPFGESTGASVIFGTTGGVIEAALRTAYEWITGETLKEVEFHGVRGLDGLKEASINIGGKEINIGVAHGLGNARKLLEEIESGESKYHAIEIMACPGGCIDGGGQPYHFGDLDIVKKRMDALYREDRNKPLRKSHENPEVQALYKEFIGDVGGKKAHDLLHTHYIKRQKL

SEQ ID NO: 29 - DNA, 1101 bp, Unknown
  Clostridium ragsdalei
atggaatgtgtggatgaaaaaggtgagatactatgtcaaaaaacatgtccttttgatgcaatttttatagacaataagaaaaattgtgcttacatagataaagaaaagtgtaccgattgtggtttgtgtgtagatgtttgccctactgggggaataatggataaagttcagttcattcctattttggatattttaaaaagtaaatctccagttgtggctatagtggctcctgccataataggacagtttggggaagatgttactatggatcaacttaggaccgcttttaaaaaactgggatttactgatatgattgaagtggcattttttgcagatatgcttactttaaaggaatctattgaatttgacaatcatgtaaaagatgaaaaagattttatgataacttcctgctgttgtcctatgtgggtggctatggtaaaaaaggtatacagtaacttggttaaacatgtatctccctctgtatctccgatggttgcaggaggaagagtacttaaaaagttaagtccttactgcaaggtagtgtttataggcccatgtattgctaaaaaatctgaggcaaaggaagaagatataaaaggagcaatagattttgtacttacttttgaagaattaagagatatatttgatgcttttcatatagttccatctaaacttgaaggagatttttcatctaaatatgcttctagaggtggaagattatatgcccgtacaggtggagtttctattgcagtaagcgaagctgtggaaaagatttttcctgaaaagcataaactatttagtgcaattcaggcaaatggcattagagaatgtaaagaaatgcttaccaaggtgcaaaatggagaaataaaagctaattttattgaaggaatgggctgtattggtggatgtgtaggtggtcccaaagcaattgcatctaaggatgaaggtagggatcgagtaaataaatttgcacaagattctgaaataaaagttgctgtagatagtgaatgtatgcatggagtattacatgctttggatatacattctatagatgattttaaggatgagaaaaaaatagaactgttagaacgagaattttaa

SEQ ID NO: 30 - protein, 366 aa, Unknown
  Clostridium ragsdalei
MECVDEKGEILCQKTCPFDAIFIDNKKNCAYIDKEKCTDCGLCVDVCPTGGIMDKVQFIPILDILKSKSPVVAIVAPAIIGQFGEDVTMDQLRTAFKKLGFTDMIEVAFFADMLTLKESIEFDNHVKDEKDFMITSCCCPMWVAMVKKVYSNLVKHVSPSVSPMVAGGRVLKKLSPYCKVVFIGPCIAKKSEAKEEDIKGAIDFVLTFEELRDIFDAFHIVPSKLEGDFSSKYASRGGRLYARTGGVSIAVSEAVEKIFPEKHKLFSAIQANGIRECKEMLTKVQNGEIKANFIEGMGCIGGCVGGPKAIASKDEGRDRVNKFAQDSEIKVAVDSECMHGVLHALDIHSIDDFKDEKKIELLEREF

SEQ ID NO: 31 - DNA, 1374 bp, Unknown
  Clostridium ragsdalei
ttgacagttaagactgaaggtattgtcaaaattgataaagagttgtgtacaggatgtaggcgatgtgcagatgtttgtcctgtagatgctatagaaggtgaaaaaggacaacctcaaaaaattaatactgaacgttgtgttttgtgtggtcagtgtgtacaaatttgcagtgcttatgcatctgcatttgatgaagatattactcctcgtgagcaaaagataaaagagcgtaatatgctcccctctgttaaagagcccttatttgcatcctactatacaggccatgccatagaagtaaaagaggccttagcaaattctaaactttttactatggttcaatgtgcaccagcagtacgtgtagctattgctgaagaatttggtatgccacttggaagtttaacaccagggaaaatggcagctgcactaagagagctaggttttgatcgaatttatgatactaattttgctgctgatctcactattatggaggaaggtaatgaacttattaaaagggttactgaaggtggagtgctgcccatgttcacttcatgttgtcctgcttgggtaaaatttattgagcaggattatccggagcttattcctcatctgtcttcttgtaaatctccacaacaaatggaaggtgctctgcttaaaacatatggtgcacaggttgatggtgtagatgctggcaagatttatagtgtttcagttatgccttgtatttgcaaaaaatttgaatgtgaacgtcctgaaatgaaagacagtggatatcaggatgtagattctgtaattaccacacgggaacttggacaattaatcaaagatgctggcattgattttaatgctttacctgaaaatgaatttgacaagccacttgggacttattctggggcaggtactattttttgcgctactggaggtgttatggaagctgccctgcgtacggcatataaattgattactaaagaagagattccagatgtcaatctcaaatttataagaggcggcgaaggagtaagaagttcagaagttaaagtaggagatctgacattaaaagtagcagtagttgctggtctgaaaaatgttgtaccagttttggaagcaattaaagctggaaaagcagatttccatttcattgaagtgatgacctgtccagttggatgtgttagtggagggggacaacctaagatattgatacctgatgaaaaaactgatgcttatactaatcgtacgtgcagtacgtatgtacatgatgaaaatatggaatatagaaaatcacatgataatcctgagatacagaaaatttataaagaattcttggtagaagataatattcatcatttgcttcatactacgtatacaccaaggaggtaa

SEQ ID NO: 32 - protein, 457 aa, Unknown
  Clostridium ragsdalei
MTVKTEGIVKIDKELCTGCRRCADVCPVDAIEGEKGQPQKINTERCVLCGQCVQICSAYASAFDEDITPREQKIKERNMLPSVKEPLFASYYTGHAIEVKEALANSKLFTMVQCAPAVRVAIAEEFGMPLGSLTPGKMAAALRELGFDRIYDTNFAADLTIMEEGNELIKRVTEGGVLPMFTSCCPAWVKFIEQDYPELIPHLSSCKSPQQMEGALLKTYGAQVDGVDAGKIYSVSVMPCICKKFECERPEMKDSGYQDVDSVITTRELGQLIKDAGIDFNALPENEFDKPLGTYSGAGTIFCATGGVMEAALRTAYKLITKEEIPDVNLKFIRGGEGVRSSEVKVGDLTLKVAVVAGLKNVVPVLEAIKAGKADFHFIEVMTCPVGCVSGGGQPKILIPDEKTDAYTNRTCSTYVHDENMEYRKSHDNPEIQKIYKEFLVEDNIHHLLHTTYTPRR

SEQ ID NO: 33 - DNA, 1200 bp, Unknown
  Clostridium autoethanogenum
gtgatagacgtacatgaagcattcaatatagtaatgaataacacaaaactgcttaaaggtgaagatatatcgttgataaattctcttaacagggtattggcagaggatataagctcaaaagataatcttcccccatttgacaaatcctgtatggatgggtatgctttaaaaagtgaagatactaaggaaaaaatgtcaaaatttcgaattaagggaagcataaaggcgggagatttttctgatatagtattgaaaaatggtgaagccataaaaataatgacaggagctccagtaccaaaaggtgcagatgcagttattcaaatagaaaaagtaaaagtagaaggaaaagaacttcatgtattagaaaatatatctcctggaaccaacatatttaaaactggtgaggagataaaaattggtgatgttgctttaagaaaaggaaagattttgagacctgcagaaatagggttattggcatcactaggttatactaaaataaaatgttataaagcccctaaaattataataataaatactggggatgaacttataaatatagatcaaaacttaatgcaaggtaaaataaggaattgtaatgaatatacattaattgcccttattaaaaatttaaatgcagaagttaaatcatatgggataataagagatgataaggataagatttttaatgctataaaaactgcatttgaagagggagatataatcataactactggaggagcatctgtaggtgattacgattttatagaagatgttcttcagaaaataggaacagatataaagtttacttcggtagctattaaaccaggaaaaccagttgtttttgcaacttttaaagataaattgttctttggacttccaggaaatccgctttcggtaataaattcatttgaaagttttgtagcaccatctattaaaaaaatgattggaagagatgatgcgtttcctgaagaatttcctgtaactttaaaagatgattttaaatcaggaaaagaaagagactgctatatgtatgtaaacataaaaaaggaagataaccgttattatgcctatgatgtaggaagacaagattccaatgggctttttacgcttactaagtcaaatggagtcgtcatcatggaaaagggaactagtatagcaaaagctggagatattttaaatggaaaatttatattcaaataa

SEQ ID NO: 34 - protein, 399 aa, Unknown
  Clostridium autoethanogenum
VIDVHEAFNIVMNNTKLLKGEDISLINSLNRVLAEDISSKDNLPPFDKSCMDGYALKSEDTKEKMSKFRIKGSIKAGDFSDIVLKNGEAIKIMTGAPVPKGADAVIQIEKVKVEGKELHVLENISPGTNIFKTGEEIKIGDVALRKGKILRPAEIGLLASLGYTKIKCYKAPKIIIINTGDELINIDQNLMQGKIRNCNEYTLIALIKNLNAEVKSYGIIRDDKDKIFNAIKTAFEEGDIIITTGGASVGDYDFIEDVLQKIGTDIKFTSVAIKPGKPVVFATFKDKLFFGLPGNPLSVINSFESFVAPSIKKMIGRDDAFPEEFPVTLKDDFKSGKERDCYMYVNIKKEDNRYYAYDVGRQDSNGLFTLTKSNGVVIMEKGTSIAKAGDILNGKFIFK

SEQ ID NO: 35 - DNA, 570 bp, Unknown
  Clostridium autoethanogenum
atggaaaatttatattcaaataagaggtcagtaatttctattatttcatctagttcaaattcgggtaagactaccttgatagaaggaataataagaattctaaaaagcagaggatataaggttggtgcaataaagaatgatgctcataagttacagatagattacccaggaaaagacagctttagatttacagaggcaggtgcggacaatgttgttattgcatcggataatacagtggctatgataaaaaaagtaagtggacccaaaagtatagaagaactactgttgctttttcaagatgtagatattgtaatagtggaaggcttcaagggtaacgaatttcctaaaatagaagtatacaggaaaaatgcaagcaaatgtttactttacaaaaattctaaatataattttcaaaattttgtagctattgtaaccaatgaaaacttaataactgatattcctgtatttgatataaatgatacaaaaaaaatagctgattttattgagaacgactttataggaggtaacaaaaatggagaaaaccatggaacttcatgtagtcaaatatga

SEQ ID NO: 36 - protein, 189 aa, Unknown
  Clostridium autoethanogenum
MENLYSNKRSVISIISSSSNSGKTTLIEGIIRILKSRGYKVGAIKNDAHKLQIDYPGKDSFRFTEAGADNVVIASDNTVAMIKKVSGPKSIEELLLLFQDVDIVIVEGFKGNEFPKIEVYRKNASKCLLYKNSKYNFQNFVAIVTNENLITDIPVFDINDTKKIADFIENDFIGGNKNGENHGTSCSQI

SEQ ID NO: 37 - DNA, 777 bp, Unknown
  Clostridium autoethanogenum
atggaacttcatgtagtcaaatatgacaaagaatgtaaaaagacagtagaggaatcaactatttgtgaatatcctttaaatgtatttgtaaatggtgaacatttgacagtactcttatgtacgcctgaaaagcttaaggaattaacaataggtttcttgacctttagaggtgttataaaatctctagatgaaataaaatctctagagatagatgaaaaaagtggagcgtccagggtaactttgaaaaatagccaatttaataaagagttgtattcaaagcaagtgcttcctataacatttagtgaaaatgagaaaagtaagttcttttcgtatattattgattccatggaaattagtataatcaacaatgataatgtttacattcatgtcgataaaatctatgatctaatgatggacaatcttggatattccaagacgtttaaactcactggaggaacacattgtgcagctctttgtgatgaagataaagtaatatctatttgtgaggatgtggctagacacaatgctgtagacaagcttataggtgaggcatttataaaaaatatttatttaaaggataaaataatatttgtgagcagcagagtatcttttgaaatggtatataaaattgctaggctaggggtacctataataatatctaaatctgcacctacaagtctttctatagaatttgcaaaagctttaaatgttacattaattggatttgtaaggggagaaagaatgaatgtatatacaaatccacagagaataatatag

SEQ ID NO: 38 - protein, 258 aa, Unknown
  Clostridium autoethanogenum
MELHVVKYDKECKKTVEESTICEYPLNVFVNGEHLTVLLCTPEKLKELTIGFLTFRGVIKSLDEIKSLEIDEKSGASRVTLKNSQFNKELYSKQVLPITFSENEKSKFFSYIIDSMEISIINNDNVYIHVDKIYDLMMDNLGYSKTFKLTGGTHCAALCDEDKVISICEDVARHNAVDKLIGEAFIKNIYLKDKIIFVSSRVSFEMVYKIARLGVPIIISKSAPTSLSIEFAKALNVTLIGFVRGERMNVYTNPQRII

SEQ ID NO: 39 - DNA, 486 bp, Unknown
  Clostridium autoethanogenum
atgttaactaaacagcaaaatgaagacctgtctggacaagatgtaattgaaaaatatcctaaagagcagagatttactcttgctatactacaggatatacagagaaagtacaaatatataccaagagaagcactggagaatttagctaagtatttggacacgcctgtaagtagactgtatggtatggctactttttataaggcattgagccttactccaaaaggggaaaacataataactgtatgtgatggaaccgcttgccatgttgctggttctatggttgtaatggatgaacttgaaaaggcaataggaattaaaccaggtgaaactacagaggatctcaaattttcaataaatacagttaactgtataggatgctgtgcaatagctcctgtcatgatgataaatgacaaatattatggaaatttaacacctaaactggttgaagaaattcttagtgagtataggagtgagagtgatgagtga

SEQ ID NO: 40 - protein, 161 aa, Unknown
  Clostridium autoethanogenum
MLTKQQNEDLSGQDVIEKYPKEQRFTLAILQDIQRKYKYIPREALENLAKYLDTPVSRLYGMATFYKALSLTPKGENIITVCDGTACHVAGSMVVMDELEKAIGIKPGETTEDLKFSINTVNCIGCCAIAPVMMINDKYYGNLTPKLVEEILSEYRSESDE

SEQ ID NO: 41 - DNA, 1800 bp, Unknown
  Clostridium autoethanogenum
atgagtgataaaaaaactgtcaatatatgttgtgggacaggttgtttagctaaaggcagtatggaagtatatgaagaaatgaaggcacaaatagctaaattaggggcaaatgcagaagtaaatgttaaattaaaagcaacaggttgcgatggattgtgtgagaaaggtcctgtactgaaaatatatccagatgacattgcatattttaaagttaaagtagaagatgtagaagacgtagtaaaaaagacattgatgaatggggaaataattgaaaaattattatattttgagactgctacaaaacagagattaagaaatcataaagaaagtgaattttgtaaaagacaatacaaaattgctctcagaaatgttggtgaaatagatccaataagtttggaagattatgttgaaagaggcggatacaaagctcttaaaaaagcaataagcagcatgaaacctgaagatgtgcttgaagaaataacaaaatcaggtcttagaggaagaggtggagcaggattcccaacaggacgtaaatggaaaactgctgcagatattgatacatcacctatatatgtagtatgtaatggtgatgaaggagatcctggagcatttatggatagaagtataatggagggagatcctaacagtgttatagaaggtatgacattatgtgcttatgcagtaggaggtacaaatggatttgcttatataagagatgaatatggacttgctgtagaaaatatgcagaaagctattaataaagcaaaagatgaaaatttattaggtaataatatattaggaactgatttttccttcgatatacagatagtaagaggtggaggagcttttgtatgtggtgaatctactgcacttatgtcgtctatagaaggtatggtaggtgaacctagagctaaatatatacacactacagaaaaaggattgtggggacaacctacagttttaaataatgtagaaacttgggccaatgtacctataataattgaaaaaggcggagattggtatcatgctataggaactatggagaagagtaagggaacaaaggtattctcattagttggaaaagttaagaatactggacttgtagaagtacctatgggaactactcttagagaaataatatatgatattggcggtggagtattaaatgatagaaagtttaaggcagttcaaataggtggaccttcaggtggatgtttaccagctgaatatttagatttgccagtagattatgatactttggttaaagcagattccatgatgggttcaggcggaatgatcgtaatggatgatagaacctgtatggtagatgtaactagatattacctgagcttcttggctgaagaatcttgtggaaagtgtgtaccttgtagagaaggcgtaaagaggatgcttgaaatactcactgacatatgcaatggtgatggaaaagaaggagacatagaagagcttctcgaaatatgttccatgacaagcaaggcatctctgtgcagtcttggtaagagtgctccaaatccagtaattgcttctataagatattttagagatgaatttgaagagcatataaagaataagagatgtagagcaggagtttgtaagaaacttactacatttggtatagacgaggataaatgtaagggatgcgatatgtgtaaaaagaattgtccagctgattgtataacaggggaaattaagaaaccacatacaatagatgctgataagtgcttgagatgcggtaactgcatgaacatctgtaagtttgatgctgttaaggttctatag

SEQ ID NO: 42 - protein, 599 aa, Unknown
  Clostridium autoethanogenum
MSDKKTVNICCGTGCLAKGSMEVYEEMKAQIAKLGANAEVNVKLKATGCDGLCEKGPVLKIYPDDIAYFKVKVEDVEDVVKKTLMNGEIIEKLLYFETATKQRLRNHKESEFCKRQYKIALRNVGEIDPISLEDYVERGGYKALKKAISSMKPEDVLEEITKSGLRGRGGAGFPTGRKWKTAADIDTSPIYVVCNGDEGDPGAFMDRSIMEGDPNSVIEGMTLCAYAVGGTNGFAYIRDEYGLAVENMQKAINKAKDENLLGNNILGTDFSFDIQIVRGGGAFVCGESTALMSSIEGMVGEPRAKYIHTTEKGLWGQPTVLNNVETWANVPIIIEKGGDWYHAIGTMEKSKGTKVFSLVGKVKNTGLVEVPMGTTLREIIYDIGGGVLNDRKFKAVQIGGPSGGCLPAEYLDLPVDYDTLVKADSMMGSGGMIVMDDRTCMVDVTRYYLSFLAEESCGKCVPCREGVKRMLEILTDICNGDGKEGDIEELLEICSMTSKASLCSLGKSAPNPVIASIRYFRDEFEEHIKNKRCRAGVCKKLTTFGIDEDKCKGCDMCKKNCPADCITGEIKKPHTIDADKCLRCGNCMNICKFDAVKVL

SEQ ID NO: 43 - DNA, 768 bp, Unknown
  Clostridium autoethanogenum
gtgaatgtagatatgaaaattacaatagatggaaaagcttgtgaagctgaaaaaggagaattcatattacaaatagcaagaagaaataacatatatatacctacattatgtcacagcgatgcattgcctgggcttgctagctgtagactatgtatagttaaagtagtagataggggacgtgcaaagatagtaacttcctgtatattccctgtaagtaaggaagtagaagttataactaatgacgatgaaataaagagaatgagaaaaaacatagttatgcttttaaaagtaagatgccctgaaaataaagaggtaaatgaattagctaaagcctttggagtagaggaaaagagagtaaagaggttcaaattggatccagaacaaaattgtgttttgtgcggactttgtgcaaaagcttgcaaggaattaggtactggagcaatttcaacagttaataggggtatgtataaagaagtagcaactccatatcacgaatcttcaccggaatgtataggatgtgcttcctgtgcaaatgtttgtccaactaatgcaataaaagttgtggataaagatggagaaagagaaatatggggcaaaaaattcaagatggttaagtgtgatttgtgcggagaatattttgctacagaagaacatgtaaaatatgcttacaataggcttggaaaagagcagccagaaaaacttatgtgtagcagctgcaagaagaaagttacagccaaagatgtcaaaaatatttttgagaacgtgtga

SEQ ID NO: 44 - protein, 255 aa, Unknown
  Clostridium autoethanogenum
VNVDMKITIDGKACEAEKGEFILQIARRNNIYIPTLCHSDALPGLASCRLCIVKVVDRGRAKIVTSCIFPVSKEVEVITNDDEIKRMRKNIVMLLKVRCPENKEVNELAKAFGVEEKRVKRFKLDPEQNCVLCGLCAKACKELGTGAISTVNRGMYKEVATPYHESSPECIGCASCANVCPTNAIKVVDKDGEREIWGKKFKMVKCDLCGEYFATEEHVKYAYNRLGKEQPEKLMCSSCKKKVTAKDVKNIFENV

SEQ ID NO: 45 - DNA, 555 bp, Unknown
  Clostridium autoethanogenum
atgaaaccagagtttaattcttttgtaatagccgatcctgacaagtgcataggctgtagatcttgtgagattgcctgtgctgcaaaacatagagaagatactcaaggaaaaaccattggaactatgaataataaagttactccaaggttattctttgttaaaaataaaggaaatgtaatgccagtacaatgcagacattgtgaggatgcaccatgtctaaatgcctgcccagttaatgctatagttgaaaaagatggaagtatcattataaatgaaagtgcatgtataggatgtcagacctgtacaatagtatgtccggtaggtgctgtaagtttactgcctagaactcaaggtaaagtagttacaggaggaattcaggttaaagtaagagcagcagcttataaatgtgatttatgtaaggaagagggaggagaacctgcttgcgtcaaagaatgtccaaaagaggccttgaggttagtagatcctagagaagataaaaaagatcgtagtgtgaaagctgctatggaactgttaaatataaacgcaaatctctaa

SEQ ID NO: 46 - protein, 184 aa, Unknown
  Clostridium autoethanogenum
MKPEFNSFVIADPDKCIGCRSCEIACAAKHREDTQGKTIGTMNNKVTPRLFFVKNKGNVMPVQCRHCEDAPCLNACPVNAIVEKDGSIIINESACIGCQTCTIVCPVGAVSLLPRTQGKVVTGGIQVKVRAAAYKCDLCKEEGGEPACVKECPKEALRLVDPREDKKDRSVKAAMELLNINANL

SEQ ID NO: 47 - DNA, 567 bp, Unknown
  Clostridium autoethanogenum
atgaagaattgcctcgtagtagcagatcctaataaatgcataggatgtaggacttgtgaagcagcttgtggtattgcacattcaggaggggacttttttaacacaaatgtatccaagattaattttaatcctcgcttaaatgtgataaaaactgctaaagtaagtgctcctgttcaatgcagacaatgcgaagatgcaccttgtggtaaagcttgtccagttaacgctatttcaaatgaaaatggttatgttagtgtaaataaagatgtatgtgttggatgtaaaatctgcatgttagcttgtccttttggagctattgaattagcttctcaatatagggatggagaagttgtagaccaaaagggacttaagatgagtgaggaaggtaatcctactgtgaatggaaaaggaagagtggtagcaaataagtgtgatctctgccaggatagggatggagggcctgcttgtatagaagtttgtcctacaaaatctctcaaactagttacttatgatgacaataataatatagttgaaaaaaaagatgacgacgaacgtgaagtaagctaa

SEQ ID NO: 48 - protein, 188 aa, Unknown
  Clostridium autoethanogenum
MKNCLVVADPNKCIGCRTCEAACGIAHSGGDFFNTNVSKINFNPRLNVIKTAKVSAPVQCRQCEDAPCGKACPVNAISNENGYVSVNKDVCVGCKICMLACPFGAIELASQYRDGEVVDQKGLKMSEEGNPTVNGKGRVVANKCDLCQDRDGGPACIEVCPTKSLKLVTYDDNNNIVEKKDDDEREVS

SEQ ID NO: 49 - DNA, 957 bp, Unknown
  Clostridium ragsdalei
gtgatagacgtacatgaagcattcaatatagtaatgaataatacaaaactgcttaaaagtgaagatatgtccctgataaattctcttaacagggtattggcagaggatataagctcaaaagataatcttcccccatttgacaaatcctgtatggatgggtatgctttaaaaagtgaagatactaaggaaaaaatgtcaaaatttcaaattaagggaagcataaaggcgggagatttttctgatatagtattaaaaaatggtgaagccataaaaataatgacaggagctccagtaccaaaaggtgcagatgcaattattcaaatagaaaaagtaaaagtagaaggaaaagaacttcatgtattggaaaaggtatctcctggaaccaacatatttaaaactggtgaggagataaaaattggtgatgttgctttaaaaaagggaaaaatcgtaagacctgcagaaatagggttattggcatcactaggttatactaaaataaaatgctacaaagtccctaaaattataataataaatacaggggatgaacttataaatatagatcaaaacttaatgcaaggtaaaataagaaattgtaatgaatacacattaattgcccttattaaaaatttaaatgcagaagttaaatcgtatgggataataagagatgataagaataaaatttttaatgctataaaaactgcatttgaagagggagatataatcataactactggaggagcatctgtgggtgattacgattttatagaagatgttcttaaggaaataggaacagatataaaatttacttcggtagctattaaaccaggaaaaccagttgtttttgcaacttttaaagataaattattctttggacttccaggaaatccactttcagtaataaattcatttgaaagttttgtagcaccatctattaaaaaaaatgattggaagagatga

SEQ ID NO: 50 - protein, 318 aa, Unknown
  Clostridium ragsdalei
MIDVHEAFNIVMNNTKLLKSEDMSLINSLNRVLAEDISSKDNLPPFDKSCMDGYALKSEDTKEKMSKFQIKGSIKAGDFSDIVLKNGEAIKIMTGAPVPKGADAIIQIEKVKVEGKELHVLEKVSPGTNIFKTGEEIKIGDVALKKGKIVRPAEIGLLASLGYTKIKCYKVPKIIIINTGDELINIDQNLMQGKIRNCNEYTLIALIKNLNAEVKSYGIIRDDKNKIFNAIKTAFEEGDIIITTGGASVGDYDFIEDVLKEIGTDIKFTSVAIKPGKPVVFATFKDKLFFGLPGNPLSVINSFESFVAPSIKKNDWKR

SEQ ID NO: 51 - DNA, 570 bp, Unknown
  Clostridium ragsdalei
atggaaaatttatattcaaataagaggtcagtaatttctattatttcatctagttcaaattcaggtaagactaccttaatagaaggaataataagaattttaaaaagcagaggatataaggttggtgcaataaagaatgatgctcataagttacagatagattatccaggaaaagacagctttagatttacagaggcaggtgcagacaatgttgttattgcatcggataatacagtggctatgataaaaaaagtaagtggaccaaaaagtatagaagaattgctgttgctttttcaggatgtagatattgtaatagtggaaggttttaagggcaacgaatttcctaaaatagaagtatacaggaaaaatgcaagtaaatgtttactctacaaaaattctgaatataattttcaaaattttgtagctattgtaaccaatgaaaatttaataactgatattcctgtatttgatataaatgatacaaaaaaagtagctgattttattgaaagcaactttataggaggtaacaaaaatggagaaaaccatggaacttcatgtagtcaaatatga

SEQ ID NO: 52 - protein, 189 aa, Unknown
  Clostridium ragsdalei
MENLYSNKRSVISIISSSSNSGKTTLIEGIIRILKSRGYKVGAIKNDAHKLQIDYPGKDSFRFTEAGADNVVIASDNTVAMIKKVSGPKSIEELLLLFQDVDIVIVEGFKGNEFPKIEVYRKNASKCLLYKNSEYNFQNFVAIVTNENLITDIPVFDINDTKKVADFIESNFIGGNKNGENHGTSCSQI

SEQ ID NO: 53 - DNA, 789 bp, Unknown
  Clostridium ragsdalei
atggagaaaaccatggaacttcatgtagtcaaatatgacaaagaatgtaaaaagacagtggaggaatcaactatttgcgaatatcctttaaatgtatttgtaaatggtgaacatttgacagtgctcttatgtactcctgaaaagcttaaggaattaacaataggtttcttggtctttaaaggtattataaaatctctagatgaaataaaatctttagagatagatgaaaaaagtggagcgtccagggtaatcttgaaaaatagacaatttaataaagagttgtattcaaagcaagtacttcctacaacatttaatgaaaatgaaaaaagtaaattcttttcatatattattgattccatgaaaattagtctaatcaataatgataatgtttacatacatgttgataaaatctatggcttaatgatggacaatcttggatattccaagacttttaaactcactggaggagcacattgtgcagctctttgtgatgaagataaagtaatatctatttgtgaggatgtggccagacacaatgctgtagacaagcttataggtgaggcatttataaaaaatatttgtttaaaagataaaataatatttgtgagtagcagggtatcttttgaaatggtatataaaattgctagacttggggtacctataataatatctaaatctgcacctacaaatctttctatagaatttgcaaaagctttaaatgttacattaattggatttgtaaggggagaaagaatgaatgtatatacaaatccacagagaataatatag

SEQ ID NO: 54 - protein, 262 aa, Unknown
  Clostridium ragsdalei
MEKTMELHVVKYDKECKKTVEESTICEYPLNVFVNGEHLTVLLCTPEKLKELTIGFLVFKGIIKSLDEIKSLEIDEKSGASRVILKNRQFNKELYSKQVLPTTFNENEKSKFFSYIIDSMKISLINNDNVYIHVDKIYGLMMDNLGYSKTFKLTGGAHCAALCDEDKVISICEDVARHNAVDKLIGEAFIKNICLKDKIIFVSSRVSFEMVYKIARLGVPIIISKSAPTNLSIEFAKALNVTLIGFVRGERMNVYTNPQRII

SEQ ID NO: 55 - DNA, 486 bp, Unknown
  Clostridium ragsdalei
atgttaactaaacagcaaaatgaagacctgtctggacaagatgtaattgaaaaatatcctaaagagcagagatttactcttgctatactacaggatatacagagaaagtacaaatatatacccagagaagcactggagaatttagctaagtatttggacacgcctgtaagtagactgtatggtatggctactttttataaggcattgagccttactccaaaaggggaaaacataataactgtatgtgatggaaccgcttgccatgttgctggttctatggttgtaatggatgaacttgaaaaggcaataggaattaaaccaggtgaaactacagaagatcttaaattttcaataaatacagttaactgtataggatgctgtgcaatagctcctgtcatgatgataaatgacaaatattttggaaatttaacacctaaactggttgaagaaattcttagtgagtataggagtgaaagccatgagtga

SEQ ID NO: 56 - protein, 161 aa, Unknown
  Clostridium ragsdalei
MLTKQQNEDLSGQDVIEKYPKEQRFTLAILQDIQRKYKYIPREALENLAKYLDTPVSRLYGMATFYKALSLTPKGENIITVCDGTACHVAGSMVVMDELEKAIGIKPGETTEDLKFSINTVNCIGCCAIAPVMMINDKYFGNLTPKLVEEILSEYRSESHE

SEQ ID NO: 57 - DNA, 1821 bp, Unknown
  Clostridium ragsdalei
gtgagtataggagtgaaagccatgagtgataaaaaaattgtcaatatatgttgtggaacaggttgcttagctaaaggcagcaaggaagtatatgaagaaatgaaggcacaaatagctaaattaggggcaaatgcagaagtaaatgttaaattaaaagcaacaggttgcgatggattgtgtgagaaaggtcctgtactgaaaatatatccagatgacattgcatattttaaagttaaagtagaagatgtagaagacgtagtaaaaaagacattgatgaatggggaaataattgaaaaattattatattttgaaactgctacaaaacagagattaagaaatcataaagaaagtgaattttgtaaaagacaatacaaaattgctctcagaaatgttggtgaaatagatccaataagtttggaagattatgttgaaagaggcggatataaagctcttaaaaaagcaataagcagcatgaaacctgaagatgtgcttgaagaaataacaaaatcaggtcttagaggaagaggtggagcaggattcccaacaggacgtaaatggaaaactgctgcagatattgatacatcacctatatatgtagtatgcaatggtgatgagggagatcctggagcatttatggatagaagtataatggagggagatcctaacagtgttatagaaggtatgacattgtgtgcctatgcagtaggaggtacaaacggctttgcttatataagagatgaatatggacttgctgtagaaaatatgcagaaagctattaataaagcaaaagatgaaaatttattaggtaataatatattaggaactgacttttccttcgatatacagatagtaagaggtggaggagcttttgtatgtggtgagtctactgcacttatgtcatctatagaaggtatggtaggagaacctagagctaaatatatacacactacagaaaaaggattgtggggacaacctactgttttaaataatgtagaaacttgggccaatgtacctataataattgaaaaaggtggagattggtatcatgctataggaactatggagaagagtaagggaacaaaagtattctcattagttggaaaagttaagaatactggacttgtagaagtacctatgggaactactcttagagaaataatatatgatattggcggtggagtattaaacgacagaaagtttaaggcagttcaaataggtggaccttcaggaggatgtttaccatctgaatatttagacttgccagtagattatgatactttggttaaagcggattctatgatgggttccggcggaatgatcgtaatggatgatagaacctgtatggtagatgtaactagatattacttgagtttcttagctgaagaatcttgtggaaagtgtgtaccttgtagagaaggcgtaaagagaatgcttgaaatactcactgatatatgcaatggtgatggaaaagaaggagacatagaagagcttcttgaaatatgttccatgacaagcaaggcatctctgtgcagtcttggtaagagtgctccaaatccagtaaaagcagctataagatattttagagatgaatttgaagaacatataaagaataagagatgtagagcaggagtttgtaagaaacttactacatttggtatagatcaagataaatgtaagggatgcgatatgtgtaaaaagaattgtccagctgattgtataacaggggaaattaagaaaccacatacaatagatgctgataagtgcttgagatgcggtaactgcatgaacatctgtaagtttgatgctgttaaggttttatag

SEQ ID NO: 58 - protein, 606 aa, Unknown
  Clostridium ragsdalei
MSIGVKAMSDKKIVNICCGTGCLAKGSKEVYEEMKAQIAKLGANAEVNVKLKATGCDGLCEKGPVLKIYPDDIAYFKVKVEDVEDVVKKTLMNGEIIEKLLYFETATKQRLRNHKESEFCKRQYKIALRNVGEIDPISLEDYVERGGYKALKKAISSMKPEDVLEEITKSGLRGRGGAGFPTGRKWKTAADIDTSPIYVVCNGDEGDPGAFMDRSIMEGDPNSVIEGMTLCAYAVGGTNGFAYIRDEYGLAVENMQKAINKAKDENLLGNNILGTDFSFDIQIVRGGGAFVCGESTALMSSIEGMVGEPRAKYIHTTEKGLWGQPTVLNNVETWANVPIIIEKGGDWYHAIGTMEKSKGTKVFSLVGKVKNTGLVEVPMGTTLREIIYDIGGGVLNDRKFKAVQIGGPSGGCLPSEYLDLPVDYDTLVKADSMMGSGGMIVMDDRTCMVDVTRYYLSFLAEESCGKCVPCREGVKRMLEILTDICNGDGKEGDIEELLEICSMTSKASLCSLGKSAPNPVKAAIRYFRDEFEEHIKNKRCRAGVCKKLTTFGIDQDKCKGCDMCKKNCPADCITGEIKKPHTIDADKCLRCGNCMNICKFDAVKVL

SEQ ID NO: 59 - DNA, 768 bp, Unknown
  Clostridium ragsdalei
gtgaatgtagatatgaaaattacaatagatggaaaagcttgtgaagctgaaaaaggagaattcatattacaaatagcaagaagaaataatatatatatacctacactgtgccacagtgatgcattgcctgggcttgctagctgtagactgtgtatagttaaagtagtagataggggacgtgcaaagatagtaacttcctgtatattccctgtaagtaaggaagtagaagttataactaatgacgatgaaataaagagaatgagaaaaaacatagttatgcttttaaaagtaagatgccctgaaaataaagaagtaaatgaattagctaaagcctttggagtagaggaaaagagagtaaagaggttcaaattggatccagaacaaaattgtgttttgtgcggactttgtgcaaaagcttgcaaggaattaggtactggagcaatctcaacagttaataggggtatgtataaagaagtagcaactccatatcacgaatcttcaccagaatgtataggatgtgcttcctgtgcaaatgtttgtccaactaatgcaataaaagttgtggataaagatggagaaagagaaatatggggcaaaaaattcaagatggttaaatgtgatttgtgcggagaatattttgctacagaagaacacgtaaaatatgcttacaataggcttggaaaagagcagccagaaaagcttatgtgcagcagctgcaagaagaaagttacagccaaagatgtcaaaaatatttttgagaacgtgtga

SEQ ID NO: 60 - protein, 255 aa, Unknown
  Clostridium ragsdalei
MNVDMKITIDGKACEAEKGEFILQIARRNNIYIPTLCHSDALPGLASCRLCIVKVVDRGRAKIVTSCIFPVSKEVEVITNDDEIKRMRKNIVMLLKVRCPENKEVNELAKAFGVEEKRVKRFKLDPEQNCVLCGLCAKACKELGTGAISTVNRGMYKEVATPYHESSPECIGCASCANVCPTNAIKVVDKDGEREIWGKKFKMVKCDLCGEYFATEEHVKYAYNRLGKEQPEKLMCSSCKKKVTAKDVKNIFENV

SEQ ID NO: 61 - DNA, 555 bp, Unknown
  Clostridium ragsdalei
atgaaaccagagtttaattcttttgtaatagccgatcctgacaagtgcataggctgtagatcttgtgagattgcctgtgctgcaaaacatagagaagatactcaaggaaaaactattggaactatgaataataaagttactccaaggttattctttgttaaaaataaaggaaatgtaatgccggtacaatgcagacattgtgaggatgcaccatgtctaaatgcctgcccagttaatgctatagttgaaaaagatggaagtatcattataaatgaaagtgcatgtatagggtgtcagacctgtacaatagtatgtccggtaggtgctgtaagtttacttcctagaactcaaggtaaagtagttacaggaggaattcaggttaaagtaagagcagcagcttataaatgtgatttatgtaaggaagagggaggagaacctgcctgcgtcaaagaatgtccaaaagaggccttaaggttagtagatcctagagaagataaaaaagatcgtagtgtgaaagctgctatggaactgttaaatataaacgcaaatctctaa

SEQ ID NO: 62 - protein, 184 aa, Unknown; identical to SEQ ID NO: 46
  Clostridium ragsdalei

SEQ ID NO: 63 - DNA, 618 bp, Unknown
  Clostridium ragsdalei
atgaattattgcacactaaatatatctcaagaaaaaaggagagttaataaaatgaagaattgcctcgtagtagcagatcctaataaatgcataggatgtaggacttgtgaagcagcttgtggtattgcacattcaggaggggacttttttaatacaaatgtatccaaaattaattttaatcctcgcttaaatgtgataaaaactgctaaagtaagtgctcctgttcaatgcagacaatgcgaagatgcaccttgtggtaaagcttgtccagttaacgctatttcaaatgaaaatggttatgttagtgtagataaagatgtatgtgttggatgtaaaatctgcatgttagcttgtccttttggagctattgaattagcttctcaatataaggatggagaagttgtagaccaaaagggacttaagatgagtgaggaaggtaatcctactgtaaatggaaaaggaagagtggtagcaaataagtgtgatctttgccaggatagggatggaggacctgcttgcatagaagtttgtcctacaaaatctctcaaattagttacttatgatgacaataataatatagttgaaaaaaaagatgacgacgaacgtgaagtaggctaa

SEQ ID NO: 64 - protein, 205 aa, Unknown
  Clostridium ragsdalei
MNYCTLNISQEKRRVNKMKNCLVVADPNKCIGCRTCEAACGIAHSGGDFFNTNVSKINFNPRLNVIKTAKVSAPVQCRQCEDAPCGKACPVNAISNENGYVSVDKDVCVGCKICMLACPFGAIELASQYKDGEVVDQKGLKMSEEGNPTVNGKGRVVANKCDLCQDRDGGPACIEVCPTKSLKLVTYDDNNNIVEKKDDDEREVG

SEQ ID NO: 65 - DNA, 10640 bp, Unknown
  Clostridium autoethanogenum
atggataaaaaagttttaactgtttgtccttactgtggcgctggttgtaatttatacttgcatgtaaagaatggcaaaataattaaagcagagcctgctaatggtaggacaaatgaaggatcactgtgtttaaaaggacactttggttgggattttttaaacgatcctaaaatattgacatctagaattaaacatccgatgataagaaaaaacggagagctagaagaggtaagctgggatgaagctattagttttacggcttcaagattgtcacaaataaaagagaaatatggacctgattccataatgggaacaggatgtgctaggggttctggaaacgaagcaaactacataatgcaaaagtttatgagggcggttattggaaccaataacgtagatcactgtgccagagtttgacatgctccttctgtagccggtctggcttacgttttaggaaatggtgctatgtcaaatggtatacatgaaatagatgatacagatttactacttatttttggatataatggagcagcttcgcatccaatagttgctaagagaatagttagggcaaaacaaaagggtgcaaaggtaatagttgtagatccacgtataacagagtctggtaggatagcagatttatggctccctataaaaaatggaacaaatatggttcttgtaaatacttttgccaacatacttataaataaacagttttataacaaacaatatgtagaagatcatactgttggttttgaagaatatagatctatagttgaaaattatactcctgaatatgcagaaaaagttactggcataccttcagaggatatagtagaagctatgaaaatgtactcaggtgctaaaaatgccatgatattatatggtatgggagtatgtcaatttgctcaagctgtagatgtagttaagggactagcttctatagcattattaactggtaattttggaagacctaatgtaggtataggacctgtaagaggccagaacaatgttcaaggtgcttgtgatatgggagcacttcctaatgtatacccaggttatcaaagtgtaactgacgatgcaattaggcaaaaatttgaaaaagcttggggtgttaaacttccaaacaaagttggttatcacctgacacaagttcctgaattaacgcttaaagaggataaaataaaggcatattatataatgggtgaagatccagttcaaagtgatcctgattctaatgaaatgagagagacactggataaaatggaacttgtaatagttcaggatatatttatgaataaaactgcactccatgcagatgtaattttaccttccacgtcttggggagaacatgaaggagtctttagttctgcagatagaggattccagagatttagaaaagctgtagaacctaagggagatgttaaaccagattgggaaataatttcaaaaattgcctgtgctatgggttataatatgcattataacaatactgaggaaatatggaatgaacttataaatttatgtccaaatttcaaaggagcaacttataagagactcgaagaattaggaggaatccaatggccttgtccatctgaaaatcatcctggaacttcttatctctacaaaggtaataaatttaatacacctactggaaaagcaaacttatttgcagcagaatggagacctcctgtagagcagacagataaagattatccactcgttctttctacagttagagaagtaggacattattctgtaagaacaatgacaggaaactgtagggcacttcagcagttagccgatgaaccaggatatgtacaagttaatccaatggatgcaaaggctaagggaataatagatggtgagcttatgagaataagttcacgaagaggttctgtggttgcccgtgcacttattactgaaagggcaaataaaggagcagtctatatgacctatcaatggtgggtaggcgcatgtaatgaacttacatctaataatctagatccagtatcaaaaactcctgaattaaagtattgtgcagtaaaaatagaagctataaaagatcagaaagaagctgaaaagtttataaaagatcaatatgatcttttaaagaaaaagatgaatgtttaatattttaatataaagatggctaaaaagaccttgattaagaggtcttttagccaaaagctttaaatcaataggagttgatagactgtgatagacgtacatgaagcattcaatatagtaatgaataacacaaaactgcttaaaggtgaagatatatcgttgataaattctcttaacagggtattggcagaggatataagctcaaaagataatcttcccccatttgacaaatcctgtatggatgggtatgctttaaaaagtgaagatactaaggaaaaaatgtcaaaatttcgaattaagggaagcataaaggcgggagatttttctgatatagtattgaaaaatggtgaagccataaaaataatgacaggagctccagtaccaaaaggtgcagatgcagttattcaaatagaaaaagtaaaagtagaaggaaaagaacttcatgtattagaaaatatatctcctggaaccaacatatttaaaactggtgaggagataaaaattggtgatgttgctttaagaaaaggaaagattttgagacctgcagaaatagggttattggcatcactaggttatactaaaataaaatgttataaagcccctaaaattataataataaatactggggatgaacttataaatatagatcaaaacttaatgcaaggtaaaataaggaattgtaatgaatatacattaattgcccttattaaaaatttaaatgcagaagttaaatcatatgggataataagagatgataaggataagatttttaatgctataaaaactgcatttgaagagggagatataatcataactactggaggagcatctgtaggtgattacgattttatagaagatgttcttcagaaaataggaacagatataaagtttacttcggtagctattaaaccaggaaaaccagttgtttttgcaacttttaaagataaattgttctttggacttccaggaaatccgctttcggtaataaattcatttgaaagttttgtagcaccatctattaaaaaaatgattggaagagatgatgcgtttcctgaagaatttcctgtaactttaaaagatgattttaaatcaggaaaagaaagagactgctatatgtatgtaaacataaaaaaggaagataaccgttattatgcctatgatgtaggaagacaagattccaatgggctttttacgcttactaagtcaaatggagtcgtcatcatggaaaagggaactagtatagcaaaagctggagatattttaaatggaaaatttatattcaaataagaggtcagtaatttctattatttcatctagttcaaattcgggtaagactaccttgatagaaggaataataagaattctaaaaagcagaggatataaggttggtgcaataaagaatgatgctcataagttacagatagattacccaggaaaagacagctttagatttacagaggcaggtgcggacaatgttgttattgcatcggataatacagtggctatgataaaaaaagtaagtggacccaaaagtatagaagaactactgttgctttttcaagatgtagatattgtaatagtggaaggcttcaagggtaacgaatttcctaaaatagaagtatacaggaaaaatgcaagcaaatgtttactttacaaaaattctaaatataattttcaaaattttgtagctattgtaaccaatgaaaacttaataactgatattcctgtatttgatataaatgatacaaaaaaaatagctgattttattgagaacgactttataggaggtaacaaaaatggagaaaaccatggaacttcatgtagtcaaatatgacaaagaatgtaaaaagacagtagaggaatcaactatttgtgaatatcctttaaatgtatttgtaaatggtgaacatttgacagtactcttatgtacgcctgaaaagcttaaggaattaacaataggtttcttgacctttagaggtgttataaaatctctagatgaaataaaatctctagagatagatgaaaaaagtggagcgtccagggtaactttgaaaaatagccaatttaataaagagttgtattcaaagcaagtgcttcctataacatttagtgaaaatgagaaaagtaagttcttttcgtatattattgattccatggaaattagtataatcaacaatgataatgtttacattcatgtcgataaaatctatgatctaatgatggacaatcttggatattccaagacgtttaaactcactggaggaacacattgtgcagctctttgtgatgaagataaagtaatatctatttgtgaggatgtggctagacacaatgctgtagacaagcttataggtgaggcatttataaaaaatatttatttaaaggataaaataatatttgtgagcagcagagtatcttttgaaatggtatataaaattgctaggctaggggtacctataataatatctaaatctgcacctacaagtctttctatagaatttgcaaaagctttaaatgttacattaattggatttgtaaggggagaaagaatgaatgtatatacaaatccacagagaataatatagtaatttctgttaacatatttttgaatataatcttaaaaaattaatcatatagttatataaaaataatataatatttaatgttaataattagtccctaattaaataggactaagtttatattttaatttttaaataaggtaattaaaataattttaaattaaatgtgttatatgttttaaaattatttcttaagtatagaggctcaaatctttggtttagagctaatatcttattccttctaatattttaagggggaaatcaattataatattcaaatgggagggtgaagtatttaatgttaactaaacagcaaaatgaagacctgtctggacaagatgtaattgaaaaatatcctaaagagcagagatttactcttgctatactacaggatatacagagaaagtacaaatatataccaagagaagcactggagaatttagctaagtatttggacacgcctgtaagtagactgtatggtatggctactttttataaggcattgagccttactccaaaaggggaaaacataataactgtatgtgatggaaccgcttgccatgttgctggttctatggttgtaatggatgaacttgaaaaggcaataggaattaaaccaggtgaaactacagaggatctcaaattttcaataaatacagttaactgtataggatgctgtgcaatagctcctgtcatgatgataaatgacaaatattatggaaatttaacacctaaactggttgaagaaattcttagtgagtataggagtgagagtgatgagtgataaaaaaactgtcaatatatgttgtgggacaggttgtttagctaaaggcagtatggaagtatatgaagaaatgaaggcacaaatagctaaattaggggcaaatgcagaagtaaatgttaaattaaaagcaacaggttgcgatggattgtgtgagaaaggtcctgtactgaaaatatatccagatgacattgcatattttaaagttaaagtagaagatgtagaagacgtagtaaaaaagacattgatgaatggggaaataattgaaaaattattatattttgagactgctacaaaacagagattaagaaatcataaagaaagtgaattttgtaaaagacaatacaaaattgctctcagaaatgttggtgaaatagatccaataagtttggaagattatgttgaaagaggcggatacaaagctcttaaaaaagcaataagcagcatgaaacctgaagatgtgcttgaagaaataacaaaatcaggtcttagaggaagaggtggagcaggattcccaacaggacgtaaatggaaaactgctgcagatattgatacatcacctatatatgtagtatgtaatggtgatgaaggagatcctggagcatttatggatagaagtataatggagggagatcctaacagtgttatagaaggtatgacattatgtgcttatgcagtaggaggtacaaatggatttgcttatataagagatgaatatggacttgctgtagaaaatatgcagaaagctattaataaagcaaaagatgaaaatttattaggtaataatatattaggaactgatttttccttcgatatacagatagtaagaggtggaggagcttttgtatgtggtgaatctactgcacttatgtcgtctatagaaggtatggtaggtgaacctagagctaaatatatacacactacagaaaaaggattgtggggacaacctacagttttaaataatgtagaaacttgggccaatgtacctataataattgaaaaaggcggagattggtatcatgctataggaactatggagaagagtaagggaacaaaggtattctcattagttggaaaagttaagaatactggacttgtagaagtacctatgggaactactcttagagaaataatatatgatattggcggtggagtattaaatgatagaaagtttaaggcagttcaaataggtggaccttcaggtggatgtttaccagctgaatatttagatttgccagtagattatgatactttggttaaagcagattccatgatgggttcaggcggaatgatcgtaatggatgatagaacctgtatggtagatgtaactagatattacctgagcttcttggctgaagaatcttgtggaaagtgtgtaccttgtagagaaggcgtaaagaggatgcttgaaatactcactgacatatgcaatggtgatggaaaagaaggagacatagaagagcttctcgaaatatgttccatgacaagcaaggcatctctgtgcagtcttggtaagagtgctccaaatccagtaattgcttctataagatattttagagatgaatttgaagagcatataaagaataagagatgtagagcaggagtttgtaagaaacttactacatttggtatagacgaggataaatgtaagggatgcgatatgtgtaaaaagaattgtccagctgattgtataacaggggaaattaagaaaccacatacaatagatgctgataagtgcttgagatgcggtaactgcatgaacatctgtaagtttgatgctgttaaggttctatagggaggtgaatgtagatatgaaaattacaatagatggaaaagcttgtgaagctgaaaaaggagaattcatattacaaatagcaagaagaaataacatatatatacctacattatgtcacagcgatgcattgcctgggcttgctagctgtagactatgtatagttaaagtagtagataggggacgtgcaaagatagtaacttcctgtatattccctgtaagtaaggaagtagaagttataactaatgacgatgaaataaagagaatgagaaaaaacatagttatgcttttaaaagtaagatgccctgaaaataaagaggtaaatgaattagctaaagcctttggagtagaggaaaagagagtaaagaggttcaaattggatccagaacaaaattgtgttttgtgcggactttgtgcaaaagcttgcaaggaattaggtactggagcaatttcaacagttaataggggtatgtataaagaagtagcaactccatatcacgaatcttcaccggaatgtataggatgtgcttcctgtgcaaatgtttgtccaactaatgcaataaaagttgtggataaagatggagaaagagaaatatggggcaaaaaattcaagatggttaagtgtgatttgtgcggagaatattttgctacagaagaacatgtaaaatatgcttacaataggcttggaaaagagcagccagaaaaacttatgtgtagcagctgcaagaagaaagttacagccaaagatgtcaaaaatatttttgagaacgtgtgaaaattaaaagaggggtggtaatttaaatgaaaccagagtttaattcttttgtaatagccgatcctgacaagtgcataggctgtagatcttgtgagattgcctgtgctgcaaaacatagagaagatactcaaggaaaaaccattggaactatgaataataaagttactccaaggttattctttgttaaaaataaaggaaatgtaatgccagtacaatgcagacattgtgaggatgcaccatgtctaaatgcctgcccagttaatgctatagttgaaaaagatggaagtatcattataaatgaaagtgcatgtataggatgtcagacctgtacaatagtatgtccggtaggtgctgtaagtttactgcctagaactcaaggtaaagtagttacaggaggaattcaggttaaagtaagagcagcagcttataaatgtgatttatgtaaggaagagggaggagaacctgcttgcgtcaaagaatgtccaaaagaggccttgaggttagtagatcctagagaagataaaaaagatcgtagtgtgaaagctgctatggaactgttaaatataaacgcaaatctctaatttataagttataaaaatccggaaaagaaaggaatgttaaatatgccaactagtacttctatgataaatatagatgaagaattatgtacaggctgcagacgatgtgcggatgtctgccctgtagatgctatagaaggtgaacagggtaaacctcagaagataaatactgaaaagtgtgttatgtgcggacaatgcattcaagtttgtaaaggctatcaatctgtatacgacgatgttcctactccagttagcaaaaggttatttgatagaggattgttaaaggaagtagatgaaccattatttgcagcatataataaaggtcaggtaaagagtgttaaagaaattttacaaaacaaagatgtatttaaaattgtgcaatgtgcacctgctgtaagagttgctataggagaggattttggaatgcctcttggaactttaagtgaaggaaaaatggcagctgcactcagaaaattaggatttgacaaagtatatgatacaaactttggtgcagatcttactataatggaagaaggtagtgagttactaaaaagagtagctgaaggcggagttttgccaatgtttacttcttgttgtccagcatgggtaaaatatgcagaacaaacatatccagaacttttacctcatctttcaagttgtaagtctccaaatcagatggctggagctatatttaaaacttatggagcagagataaataaggttaatccggctaaaatttataatgtatctgttatgccatgtacatgcaaggaatttgaaagtgaaagagaagaaatgcatgacagtggacacagggatgtagatgcagttataactacaagggaattagcacaactgttcaaagatgctgatatagattttaatactattgaagaagaacagtttgatactcctcttggtatgtataccggtgcaggaactatatttggtgctacaggtggagttatggaagcagcacttagaactggatatgaactttatactaaaaaaactattccaagtatagatcttactatggtaagaggtggagaaggttttagaactgctgaagtagatttaggggatattagactaaaagtaggagtagtttccggcttaaaaaatgtaaaagacgttatggaatcagtaaaggcaggcaaatgtgatttgcactttatagaggttatgacctgtcctcaaggatgtataagtggtggaggacaacctaaagttatacttgattcagataaagaggaagcttataataataggaaaaagggactatataatcatgacgctaatcttacttatagaaaatcacatgaaaatccagaaataaagaaaatatatgatgagttcttagacaaaccattaggagctaagtctcatgaattattgcacactaaatatatctcaagaaaaaaggagagttaataaaatgaagaattgcctcgtagtagcagatcctaataaatgcataggatgtaggacttgtgaagcagcttgtggtattgcacattcaggaggggacttttttaacacaaatgtatccaagattaattttaatcctcgcttaaatgtgataaaaactgctaaagtaagtgctcctgttcaatgcagacaatgcgaagatgcaccttgtggtaaagcttgtccagttaacgctatttcaaatgaaaatggttatgttagtgtaaataaagatgtatgtgttggatgtaaaatctgcatgttagcttgtccttttggagctattgaattagcttctcaatatagggatggagaagttgtagaccaaaagggacttaagatgagtgaggaaggtaatcctactgtgaatggaaaaggaagagtggtagcaaataagtgtgatctctgccaggatagggatggagggcctgcttgtatagaagtttgtcctacaaaatctctcaaactagttacttatgatgacaataataatatagttgaaaaaaaagatgacgacgaacgtgaagtaagctaa

SEQ ID NO: 66 - DNA, 10640 bp, Unknown
  Clostridium ljungdahlii
atggataaaaaagttttaactgtttgtccttactgtggcgctggttgtaatttatacttgcatgtaaagaatggcaaaataattaaagcagagcctgctaatggtaggacaaatgaaggatcactgtgtttaaaaggacactttggttgggattttttaaacgatcctaaaatattgacatctagaattaaacatccgatgataagaaaaaacggagagctagaagaggtaagctgggatgaagctattagttttacggcttcaagattgtcacaaataaaagagaaatatggacctgattccataatgggaacaggatgtgctaggggttctggaaacgaagcaaactacataatgcaaaagtttatgagggcggttattggaaccaataacgtagatcactgtgccagagtttgacatgctccttctgtagccggtctggcttacgttttaggaaatggtgctatgtcaaatggtatacatgaaatagatgatacagatttactacttatttttggatataatggagcagcttcgcatccaatagttgctaagagaatagttagggcaaaacaaaagggtgcaaaggtaatagttgtagatccacgtataacagagtctggtaggatagcagatttatggctccctataaaaaatggaacaaatatggttcttgtaaatacttttgccaacatacttataaataaacagttttataacaaacaatatgtagaagatcatactgttggttttgaagaatatagatctatagttgaaaattatactcctgaatatgcagaaaaagttactggcataccttcagaggatatagtagaagctatgaaaatgtactcaggtgctaaaaatgccatgatattatatggtatgggagtatgtcaatttgctcaagctgtagatgtagttaagggactagcttctatagcattattaactggtaattttggaagacctaatgtaggtataggacctgtaagaggccagaacaatgttcaaggtgcttgtgatatgggagcacttcctaatgtatacccaggttatcaaagtgtaactgacgatgcaattagggaaaaatttgaaaaagcttggggtgttaaacttccaaacaaagttggttatcacctgacacaagttcctgaattaacgcttaaagaggataaaataaaggcatattatataatgggtgaagatccagttcaaagtgatcctgattctaatgaaatgagagagacactggataaaatggaacttgtaatagttcaggatatatttatgaataaaactgcactccatgcagatgtaattttaccttccacgtcttggggagaacatgaaggagtctttagttctgcagatagaggattccagagatttagaaaagctgtagaacctaagggagatgttaaaccagattgggaaataatttcaaaaattgcctgtgctatgggttataatatgcattataacaatactgaggaaatatggaatgaacttataaatttatgtccaaatttcaaaggagcaacttataagagactcgaagaattaggaggaatccaatggccttgtccatctgaaaatcatcctggaacttcttatctctacaaaggtaataaatttaatacacctactggaaaagcaaacttatttgcagcagaatggagacctcctgtagagcagacagataaagattatccacttgttctttctacagttagagaagtaggacattattctgtaagaacaatgacaggaaactgtagggcacttcagcagttagccgatgaaccaggatatgtacaagttaatccaatggatgcaaaggctaagggaataatagatggtgagcttatgagaataagttcacgaagaggttctgtggttgcccgtgcacttattactgaaagggcaaataaaggagcagtctatatgacctatcaatggtgggtaggcgcatgtaatgaacttacatctaataatctagatccagtatcaaaaactcctgaattaaagtattgtgcagtaaaaatagaagctataaaagatcagaaagaagctgaaaagtttataaaagatcaatatgatcttttaaagaaaaagatgaatgtttaatattttaatataaagatggctaaaaagaccttgattaagaggtcttttagccaaaagctttaaatcaataggagttgatagactgtgatagacgtacatgaagcattcaatatagtaatgaataacacaaaactgcttaaaggtgaagatatatcgttgataaattctcttaacagggtattggcagaggatataagctcaaaagataatcttcccccatttgacaaatcctgtatggatgggtatgctttaaaaagtgaagatactaaggaaaaaatgtcaaaatttcgaattaagggaagcataaaggcgggagatttttctgatatagtattgaaaaatggtgaagccataaaaataatgacaggagctccagtaccaaaaggtgcagatgcagttattcaaatagaaaaagtaaaagtagaaggaaaagaacttcatgtattagaaaatgtatctcctggaaccaacatatttaaaactggtgaggagataaaaattggtgatgttgctttaagaaaaggaaagattttgagacctgcagaaatagggttattggcatcactaggttatactaaaataaaatgttataaagcccctaaaattataataataaatactggggatgaacttataaatatagatcaaaacttaatgcaaggtaaaataaggaattgtaatgaatatacattaattgcccttattaaaaatttaaatgcagaagttaaatcatatgggataataagagatgataaggataagatttttaatgctataaaaactgcatttgaagagggagatataatcataactactggaggagcatctgtaggtgattacgattttatagaagatgttcttcagaaaataggaacagatataaagtttacttcggtagctattaaaccaggaaaaccagttgtttttgcaacttttaaagataaattgttctttggacttccaggaaatccgctttcggtaataaattcatttgaaagttttgtagcaccatctattaaaaaaatgattggaagagatgatgcgtttcctgaagaatttcctgtaactttaaaagatgattttaaatcaggaaaagaaagagactgctatatgtatgtaaacataaaaaaggaagataaccgttattatgcctatgatgtaggaagacaagattccaatgggctttttacgcttactaagtcaaatggagtcgtcatcatggaaaagggaactagtatagcaaaagctggagatattttaaatggaaaatttatattcaaataagaggtcagtaatttctattatttcatctagttcaaattcgggtaagactaccttgatagaaggaataataagaattctaaaaagcagaggatataaggttggtgcaataaagaatgatgctcataagttacagatagattacccaggaaaagacagctttagatttacagaggcaggtgcggacaatgttgttattgcatcggataatacagtggctatgataaaaaaagtaagtggacccaaaagtatagaagaactactgttgctttttcaagatgtagatattgtaatagtggaaggcttcaagggtaacgaatttcctaaaatagaagtatacaggaaaaatacaagcaaatgtttactttacaaaaattctaaatataattttcaaaattttgtagctattgtaaccaatgaaaacttaataactgatattcctgtatttgatataaatgatacaaaaaaaatagctgattttattgagaacgactttataggaggtaacaaaaatggagaaaaccatggaacttcatgtagtcaaatatgacaaagaatgtaaaaagacagtagaggaatcaactatttgtgaatatcctttaaatgtatttgtaaatggtgaacatttgacagtactcttatgtacgcctgaaaagcttaaggaattaacaataggtttcttgacctttagaggtgttataaaatctctagatgaaataaaatctctagagatagatgaaaaaagtggagcgtccagggtaactttgaaaaatagccaatttaataaagagttgtattcaaagcaagtgcttcctataacatttaatgaaaatgagaaaagtaagttcttttcgtatattattgattccatggaaattagtataatcaacaatgataatgtttacattcatgtcgataaaatctatgatctaatgatggacaatcttggatattccaagacgtttaaactcactggaggaacacattgtgcagctctttgtgatgaagataaagtaatatctatttgtgaggatgtggctagacacaatgctgtagacaagcttataggtgaggcatttataaaaaatatttatttaaaggataaaataatatttgtgagcagcagagtatcttttgaaatggtatataaaattgctaggctaggggtacctataataatatctaaatctgcacctacaagtctttctatagaatttgcaaaagctttaaatgttacattaattggatttgtaaggggagaaagaatgaatgtatatacaaatccacagagaataatatagtaatttctgttaacatatttttgaatataatcttaaaaaattaatcatatagttatataaaaataatataatatttaatgttaataattagtccctaattaaataggactaagtttatattttaatttttaaataaggtaattaaaataattttaaattaaatgtgttatatgttttaaaattatttcttaagtatagaggctcaaatctttggtttagagctaatatcttattccttctaatattttaagggggaaatcaattataatattcaaatgggagggtgaagtatttaatgttaactaaacagcaaaatgaagacctgtctggacaagatgtaattgaaaaatatcctaaagagcagagatttactcttgctatactacaggatatacagagaaagtacaaatatataccaagagaagcactggagaatttagctaagtatttggacacgcctgtaagtagactgtatggtatggctactttttataaggcattgagccttactccaaaaggggaaaacataataactgtatgtgatggaaccgcttgccatgttgctggttctatggttgtaatggatgaacttgaaaaggcaataggaattaaaccaggtgaaactacagaggatctcaaattttcaataaatacagttaactgtataggatgctgtgcaatagctcctgtcatgatgataaatgacaaatattatggaaatttaacacctaaactggttgaagaaattcttagtgagtataggagtgagagtgatgagtgataaaaaaactgtcaatatatgttgtgggacaggttgtttagctaaaggcagtatggaagtatatgaagaaatgaaggcacaaatagctaaattaggggcaaatgcagaagtaaatgttaaattaaaagcaacaggttgcgatggattgtgtgagaaaggtcctgtactgaaaatatatccagatgacattgcatattttaaagttaaagtagaagatgtagaagacgtagtaaaaaagacattgatgaatggggaaataattgaaaaattattatattttgagactgctacaaaacagagattaagaaatcataaagaaagtgaattttgtaaaagacaatacaaaattgctctcagaaatgttggtgaaatagatccaataagtttggaagattatgttgaaagaggcggatacaaagctcttaaaaaagcaataagcagcatgaaacctgaagatgtgcttgaagaaataacaaaatcaggtcttagaggaagaggtggagcaggattcccaacaggacgtaaatggaaaactgctgcagatattgatacatcacctatatatgtagtatgtaatggtgatgaaggagatcctggagcatttatggatagaagtataatggagggagatcctaacagtgttatagaaggtatgacattatgtgcttatgcagtaggaggtacaaatggatttgcttatataagagatgaatatggacttgctgtagaaaatatgcagaaagctattaataaagcaaaagatgaaaatttattaggtaataatatattaggaactgatttttccttcgatatacagatagtaagaggtggaggagcttttgtatgtggtgaatctactgcacttatgtcgtctatagaaggtatggtaggtgaacctagagctaaatatatacacactacagaaaaaggattgtggggacaacctacagttttaaataatgtagaaacttgggccaatgtacctataataattgaaaaaggcggagattggtatcatgctataggaactatggagaagagtaagggaacaaaggtattctcattagttggaaaagttaagaatactggacttgtagaagtacctatgggaactactcttagagaaataatatatgatattggcggtggagtattaaatgatagaaagtttaaggcagttcaaataggtggaccttcaggtggatgtttaccagctgaatatttagatttgccagtagattatgatactttggttaaagcagattccatgatgggttcaggcggaatgatcgtaatggatgatagaacctgtatggtagatgtaactagatattacttgagcttcttggctgaagaatcttgtggaaagtgtgtaccttgtagagaaggcgtaaagaggatgcttgaaatactcactgacatatgcaatggtgatggaaaagaaggagacatagaagagcttcttgaaatatgttccatgacaagcaaggcatctctgtgcagtcttggtaagagtgctccaaatccagtaattgcttctataagatattttagagatgagtttgaagagcatataaagaataagagatgtagagcaggagtttgtaagaaacttactacatttggtatagacgaggataaatgtaagggatgcgatatgtgtaaaaagaattgtccagctgattgtataacaggggaaattaagaaaccacatacaatagatgctgataagtgcttgagatgcggtaactgcatgaacatctgtaagtttgatgctgttaaggttctatagggaggtgaatgtagatatgaaaattacaatagatggaaaagcttgtgaagctgaaaaaggagaattcatattacaaatagcaagaagaaataacatatatatacctacattatgtcacagcgatgcattgcctgggcttgctagctgtagactatgtatagttaaagtagtagataggggacgtgcaaagatagtaacttcctgtatattccctgtaagtaaggaagtagaagttataactaatgacgatgaaataaagagaatgagaaaaaacatagttatgcttttaaaagtaagatgccctgaaaataaagaggtaaatgaattagctaaagcctttggagtagaggaaaagagagtaaagaggttcaaattggatccagaacaaaattgtgttttgtgcggactttgtgcaaaagcttgcaaggaattaggtactggagcaatttcaacagttaataggggtatgtataaagaagtagcaactccatatcacgaatcttcaccggaatgtataggatgtgcttcctgtgcaaatgtttgtccaactaatgcaataaaagttgtggataaagatggagaaagagaaatatggggcaaaaaattcaagatggttaagtgtgatttgtgcggagaatattttgctacagaagaacatgtaaaatatgcttacaataggcttggaaaagagcagccagaaaaacttatgtgcagcagctgcaagaagaaaattacagccaaagatgtcaaaaatatttttgagaacgtgtgaaaattaaaagaggggtggtaatttaaatgaaaccagagtttaattcttttgtaatagccgatcctgacaagtgcataggctgtagatcttgtgagattgcctgtgctgcaaaacatagagaagatactcaaggaaaaaccattggaactatgaataataaagttactccaaggttattctttgttaaaaataaaggaaatgtaatgccagtacaatgcagacattgtgaggatgcaccatgtctaaatgcctgcccagttaatgctatagttgaaaaagatggaagtatcattataaatgaaagtgcatgtataggatgccagacctgtacaatagtatgtccggtaggtgctgtaagtttactgcctagaactcaaggtaaagtagttacaggaggaattcaggttaaagtaagagcagcagcttataaatgtgatttatgtaaggaagagggaggagaacctgcttgcgtcaaagaatgtccaaaagaggccttgaggttagtagatcctagagaagataaaaaagatcgtagtgtgaaagctgctatggaactgttaaatataaacgcaaatctctaatttataagttataaaaatccggaaaagaaaggaatgttaaatatgccaactagtacttctatgataaatatagatgaagaattatgtacaggctgcagacgatgtgcggatgtctgccctgtagatgctatagaaggtgaacagggtaaacctcagaagataaatactgaaaagtgtgttatgtgcggacaatgcattcaagtttgtaaaggctatcaatctgtatacgacgatgttcctactccagttagcaaaaggttatttgatagaggattgttaaaggaagtagatgaaccattatttgcagcatataataaaggtcaggcaaagagtgttaaagaaattttacaaaacaaagatgtatttaaaattgtgcaatgtgcacctgctgtaagagttgctataggagaggattttggaatgcctcttggaactttaagtgaaggaaaaatggcagctgcactcagaaaattaggatttgacaaagtatatgatacaaactttggtgcagatcttactataatggaagaaggtagtgagttactaaaaagagtagctgaaggcggagttttgccaatgtttacttcttgttgtccagcatgggtaaaatatgcagaacaaacatatccagaacttttacctcatctttcaagttgtaagtctccaaatcagatggctggagctatatttaaaacttatggagcagagataaataaggttaatccggctaaaatttataatgtatctgttatgccatgtacatgcaaggaatttgaaagtgaaagagaagaaatgcatgacagtggacacagggatgtagatgcagttataactacaagggaattagcacaactgttcaaagatgctgatatagattttaatactattgaagaagaacagtttgatactcctcttggtatgtataccggtgcaggaactatatttggtgctacaggtggagttatggaagcagcacttagaactggatatgaactttatactaaaaaaactattccaagtatagatcttactatggtaagaggtggagaaggttttagaactgctgaagtagatttaggggatattagactaaaagtaggagtagtttccggcttaaaaaatgtaaaagacgttatggaatcagtaaaggcaggcaaatgtgatttgcactttatagaggttatgacctgtcctcaaggatgtataagtggtggaggacaacctaaagttatacttgattcagataaagaggaagcttataataataggaaaaagggactatataatcatgacgctaatcttacttatagaaaatcacatgaaaatccagaaataaagaaaatatatgatgagttcttagacaaaccattaggagctaagtctcatgaattattgcacactaaatatatctcaagaaaaaaggagagttaataaaatgaagaattgcctcgtagtagcagatcctaataaatgcataggatgtaggacttgtgaagcagcttgtggtattgcacattcaggaggggacttttttaacacaaatgtatccaagattaattttaatcctcgcttaaatgtgataaaaactgctaaagtaagtgctcctgttcaatgcagacaatgcgaagatgcaccttgtggtaaagcttgtccagttaacgctatttcaaatgaaaatggttatgttagtgtaaataaagatgtatgtgttggatgtaaaatctgcatgttagcttgtccttttggagctattgaattagcttctcaatatagggatggagaagttgtagaccaaaagggacttaagatgagtgaggaaggtaatcctactgtgaatggaaaaggaagagtggtagcaaataagtgtgatctctgccaggatagggatggagggcctgcttgtatagaagtttgtcctacaaaatctctcaaactagttacttatgatgacaataataatatagttgaaaaaaaagatgacgacgaacgtgaagtaagctaa

SEQ ID NO: 67 - DNA, 10633 bp, Unknown
  Clostridium ragsdalei
atggataaaaaagttttaactgtttgtccttactgcggtgctggttgtaagttatacttgcatgtaaaggatggcaagataattaaagcagagcctgctaatggtaggacaaatgaagggtccttgtgtttaaaaggacgatttggctgggattttctaaatgatcctaaaatattgacatctagaattaaacatccaatgataagaaaaaatggagagttagaagaggtaagttgggatgaagctattagttttacggcttcaaaattgtcacaaataaaagagaaatatggacctgattctataatgggaacaggatgtgctaggggttctggaaatgaagcaaactacgtaatgcaaaagtttatgagggcggttattggaaccaataacgtagatcactgtgccagagtttgacatgctccttctgtagccggtctggcttacgttttaggaaatggtgctatgtcaaatggtatacatgaaatagatgatacagatttactacttatttttggatataatggagcagcttcgcatccaatagttgctaagagaatagttagggcaaaacaaaaaggtgcaaaggtaatagttgtagatccacgtataacagagtctggtaggatagcagatttatggctccctataaaaaatggaacaaatatggttcttgtaaatacttttgccaatatacttataaacaagcaattttatgacaaacaatatgtagaagatcatactgttggttttgaagaatataaatctatagttgaggattatacgcctgaatatgcagaaaaagttactggtatacctgcagaggatatagtagaagctatgaaaatgtactccagtgctaaaaatgctatgatattgtacggtatgggagtatgtcagtttgctcaagctgtagatgtagtaaaagggttagcttcaatagctttattaactggtaattttggaagacctaatgtaggcataggacctgtaagaggccagaacaatgtgcaaggtgcctgcgatatgggagcacttcctaatgtatacccaggttatcaaagtgtaactgacgatgcaattagagaaaaatttgaaaaagcttggggagttaaactttcaaacaaagttggttatcacctgacacgagttcctgaattaacgcttaaagaggataaaataaaagcatattatataatgggcgaagatccagctcaaagtgatcctgattctaatgaaatgagggaaacacttgataaaatggaacttgtaatagttcaagatatatttatgaataaaactgcactccatgcagatgtaattttaccttctacgtcttggggagaacatgaaggagtcttcagttctgctgatagaggattccagagatttagaaaagctgtagaacctaagggcgatgttaaaccagattgggagataatttcagaaattgcatgtgctatgggttatgatatgcattataacaatactgaggaaatatgggatgaacttataaatttatgcccaaatttcaaaggagcaacttataagagattggatgaattaggaggaattcaatggccttgtccatctgaagatcatccaggaacttcttatctctacaaaggaaataaatttaatacacctactggaaaagcaaatttatttgcagcagaatggagacctcctatagagaagacagatgaagaatatccacttgttctttctacagttagagaagtagggcattactccgtaagaacaatgacaggaaactgtagggcactccagcagttagctgatgaaccaggatatgtacaaattaatccagtggatgcaaaggctaaaaaaataatagatggtgagcttatgagagtaagttcacgaagaggttctgtagttgcccgtgcacttgttactgaaagggcaaataaaggagcagtttatatgacctatcaatggtgggtaggtgcatgtaatgagcttacagctaataatttagatccagtatcaaaaactcctgaattaaagtattgtgcagtgaaggtagaagctatagaagatcagaaagaagctgaaaagtttataaaagatcaatatgcttcaataaagaaaaagatgaatgtttaatataaagatggctaaaaagaccttgattaaaaggtcttttagccaaaagctttaaatcaataggagttgatagactgtgatagacgtacatgaagcattcaatatagtaatgaataatacaaaactgcttaaaagtgaagatatgtccctgataaattctcttaacagggtattggcagaggatataagctcaaaagataatcttcccccatttgacaaatcctgtatggatgggtatgctttaaaaagtgaagatactaaggaaaaaatgtcaaaatttcaaattaagggaagcataaaggcgggagatttttctgatatagtattaaaaaatggtgaagccataaaaataatgacaggagctccagtaccaaaaggtgcagatgcaattattcaaatagaaaaagtaaaagtagaaggaaaagaacttcatgtattggaaaaggtatctcctggaaccaacatatttaaaactggtgaggagataaaaattggtgatgttgctttaaaaaagggaaaaatcgtaagacctgcagaaatagggttattggcatcactaggttatactaaaataaaatgctacaaagtccctaaaattataataataaatacaggggatgaacttataaatatagatcaaaacttaatgcaaggtaaaataagaaattgtaatgaatacacattaattgcccttattaaaaatttaaatgcagaagttaaatcgtatgggataataagagatgataagaataaaatttttaatgctataaaaactgcatttgaagagggagatataatcataactactggaggagcatctgtgggtgattacgattttatagaagatgttcttaaggaaataggaacagatataaaatttacttcggtagctattaaaccaggaaaaccagttgtttttgcaacttttaaagataaattattctttggacttccaggaaatccactttcagtaataaattcatttgaaagttttgtagcaccatctattaaaaaaaatgattggaagagatgatgcatttcctgaagaatttcctgtaactttaaaagatgattttaagtcaggaaaagaaagagactgttatatgtatgtagatataaaaaaggaagataaccattattatgcttatgatgtaggaagacaagattccaatggcctttttacacttactaagtcaaatggcgtggttatcatgaaaaagggaactagtatagcaaaagctggagatattttaaatggaaaatttatattcaaataagaggtcagtaatttctattatttcatctagttcaaattcaggtaagactaccttaatagaaggaataataagaattttaaaaagcagaggatataaggttggtgcaataaagaatgatgctcataagttacagatagattatccaggaaaagacagctttagatttacagaggcaggtgcagacaatgttgttattgcatcggataatacagtggctatgataaaaaaagtaagtggaccaaaaagtatagaagaattgctgttgctttttcaggatgtagatattgtaatagtggaaggttttaagggcaacgaatttcctaaaatagaagtatacaggaaaaatgcaagtaaatgtttactctacaaaaattctgaatataattttcaaaattttgtagctattgtaaccaatgaaaatttaataactgatattcctgtatttgatataaatgatacaaaaaaagtagctgattttattgaaagcaactttataggaggtaacaaaaatggagaaaaccatggaacttcatgtagtcaaatatgacaaagaatgtaaaaagacagtggaggaatcaactatttgcgaatatcctttaaatgtatttgtaaatggtgaacatttgacagtgctcttatgtactcctgaaaagcttaaggaattaacaataggtttcttggtctttaaaggtattataaaatctctagatgaaataaaatctttagagatagatgaaaaaagtggagcgtccagggtaatcttgaaaaatagacaatttaataaagagttgtattcaaagcaagtacttcctacaacatttaatgaaaatgaaaaaagtaaattcttttcatatattattgattccatgaaaattagtctaatcaataatgataatgtttacatacatgttgataaaatctatggcttaatgatggacaatcttggatattccaagacttttaaactcactggaggagcacattgtgcagctctttgtgatgaagataaagtaatatctatttgtgaggatgtggccagacacaatgctgtagacaagcttataggtgaggcatttataaaaaatatttgtttaaaagataaaataatatttgtgagtagcagggtatcttttgaaatggtatataaaattgctagacttggggtacctataataatatctaaatctgcacctacaaatctttctatagaatttgcaaaagctttaaatgttacattaattggatttgtaaggggagaaagaatgaatgtatatacaaatccacagagaataatatagtaatttctgataatacatttttgaatataatcttaaaaaattagtcatatagttatataaaaataatataatatttaatgttgataattagttcttaattaaataggactaaatttatattttaatttttaaataaggtaattaaaataattttaaattaaatatgttatatgttttaaaattatttcttaagcatagaggctcaaatctttgatttagagctaatatcttattccttctaatattttaagggggaaatcaattataatattcaaatgggagggtgaagtatttaatgttaactaaacagcaaaatgaagacctgtctggacaagatgtaattgaaaaatatcctaaagagcagagatttactcttgctatactacaggatatacagagaaagtacaaatatatacccagagaagcactggagaatttagctaagtatttggacacgcctgtaagtagactgtatggtatggctactttttataaggcattgagccttactccaaaaggggaaaacataataactgtatgtgatggaaccgcttgccatgttgctggttctatggttgtaatggatgaacttgaaaaggcaataggaattaaaccaggtgaaactacagaagatcttaaattttcaataaatacagttaactgtataggatgctgtgcaatagctcctgtcatgatgataaatgacaaatattttggaaatttaacacctaaactggttgaagaaattcttagtgagtataggagtgaaagccatgagtgataaaaaaattgtcaatatatgttgtggaacaggttgcttagctaaaggcagcaaggaagtatatgaagaaatgaaggcacaaatagctaaattaggggcaaatgcagaagtaaatgttaaattaaaagcaacaggttgcgatggattgtgtgagaaaggtcctgtactgaaaatatatccagatgacattgcatattttaaagttaaagtagaagatgtagaagacgtagtaaaaaagacattgatgaatggggaaataattgaaaaattattatattttgaaactgctacaaaacagagattaagaaatcataaagaaagtgaattttgtaaaagacaatacaaaattgctctcagaaatgttggtgaaatagatccaataagtttggaagattatgttgaaagaggcggatataaagctcttaaaaaagcaataagcagcatgaaacctgaagatgtgcttgaagaaataacaaaatcaggtcttagaggaagaggtggagcaggattcccaacaggacgtaaatggaaaactgctgcagatattgatacatcacctatatatgtagtatgcaatggtgatgagggagatcctggagcatttatggatagaagtataatggagggagatcctaacagtgttatagaaggtatgacattgtgtgcctatgcagtaggaggtacaaacggctttgcttatataagagatgaatatggacttgctgtagaaaatatgcagaaagctattaataaagcaaaagatgaaaatttattaggtaataatatattaggaactgacttttccttcgatatacagatagtaagaggtggaggagcttttgtatgtggtgagtctactgcacttatgtcatctatagaaggtatggtaggagaacctagagctaaatatatacacactacagaaaaaggattgtggggacaacctactgttttaaataatgtagaaacttgggccaatgtacctataataattgaaaaaggtggagattggtatcatgctataggaactatggagaagagtaagggaacaaaagtattctcattagttggaaaagttaagaatactggacttgtagaagtacctatgggaactactcttagagaaataatatatgatattggcggtggagtattaaacgacagaaagtttaaggcagttcaaataggtggaccttcaggaggatgtttaccatctgaatatttagacttgccagtagattatgatactttggttaaagcggattctatgatgggttccggcggaatgatcgtaatggatgatagaacctgtatggtagatgtaactagatattacttgagtttcttagctgaagaatcttgtggaaagtgtgtaccttgtagagaaggcgtaaagagaatgcttgaaatactcactgatatatgcaatggtgatggaaaagaaggagacatagaagagcttcttgaaatatgttccatgacaagcaaggcatctctgtgcagtcttggtaagagtgctccaaatccagtaaaagcagctataagatattttagagatgaatttgaagaacatataaagaataagagatgtagagcaggagtttgtaagaaacttactacatttggtatagatcaagataaatgtaagggatgcgatatgtgtaaaaagaattgtccagctgattgtataacaggggaaattaagaaaccacatacaatagatgctgataagtgcttgagatgcggtaactgcatgaacatctgtaagtttgatgctgttaaggttttatagggaggtgaatgtagatatgaaaattacaatagatggaaaagcttgtgaagctgaaaaaggagaattcatattacaaatagcaagaagaaataatatatatatacctacactgtgccacagtgatgcattgcctgggcttgctagctgtagactgtgtatagttaaagtagtagataggggacgtgcaaagatagtaacttcctgtatattccctgtaagtaaggaagtagaagttataactaatgacgatgaaataaagagaatgagaaaaaacatagttatgcttttaaaagtaagatgccctgaaaataaagaagtaaatgaattagctaaagcctttggagtagaggaaaagagagtaaagaggttcaaattggatccagaacaaaattgtgttttgtgcggactttgtgcaaaagcttgcaaggaattaggtactggagcaatctcaacagttaataggggtatgtataaagaagtagcaactccatatcacgaatcttcaccagaatgtataggatgtgcttcctgtgcaaatgtttgtccaactaatgcaataaaagttgtggataaagatggagaaagagaaatatggggcaaaaaattcaagatggttaaatgtgatttgtgcggagaatattttgctacagaagaacacgtaaaatatgcttacaataggcttggaaaagagcagccagaaaagcttatgtgcagcagctgcaagaagaaagttacagccaaagatgtcaaaaatatttttgagaacgtgtgaaaattaaaagaggggtggtaatttaaatgaaaccagagtttaattcttttgtaatagccgatcctgacaagtgcataggctgtagatcttgtgagattgcctgtgctgcaaaacatagagaagatactcaaggaaaaactattggaactatgaataataaagttactccaaggttattctttgttaaaaataaaggaaatgtaatgccggtacaatgcagacattgtgaggatgcaccatgtctaaatgcctgcccagttaatgctatagttgaaaaagatggaagtatcattataaatgaaagtgcatgtatagggtgtcagacctgtacaatagtatgtccggtaggtgctgtaagtttacttcctagaactcaaggtaaagtagttacaggaggaattcaggttaaagtaagagcagcagcttataaatgtgatttatgtaaggaagagggaggagaacctgcctgcgtcaaagaatgtccaaaagaggccttaaggttagtagatcctagagaagataaaaaagatcgtagtgtgaaagctgctatggaactgttaaatataaacgcaaatctctaatttataagttataaaaatccggaaaagaaaggaatgttaaatatgccaactagtacttctatgataaatatagatgaagaattatgtacaggctgcagacgatgtgcggatgtctgccctgtagatgctatagaaggtgaacagggtaaacctcagaagataaatactgaaaagtgtgttatgtgcggacaatgcattcaagtttgtaaaggctatcaatctgtatacgatgatattcctactccagttagcaaaaggttatttgatagaggattgttaaaggaagtagatgaaccattatttgcagcatataataaaggtcaggcaaagagagttaaagaaattttacaaaacaaagatgtatttaaaattgtgcaatgtgcacctgctgtaagagttgctataggagaggattttggaatgcctcttggaactttaagtgaaggaaaaatggcagctgcactcagaaaattaggatttgacaaagtatatgatacaaactttggtgcagatcttactataatggaagaaggtagtgagttactaaaaagagtagctgaaggtggagttttgccaatgtttacttcttgttgtccagcatgggtaaaatatgcagaacaaacatatccagaacttttacctcatctttcaagttgtaagtctccaaatcagatggctggagctatatttaaaacttatggagcagagataaataaggttaatccggctaaaatttataatgtatctgttatgccatgtacatgcaaggaatttgaaagtgaaagagaagaaatgcatgacagtggacacagagatgtagatgcagttataactacaagggaattagcacaactgttcaaagatgctgatatagattttaatactattgaagaagaacagtttgatactcctcttggtatgtatactggtgcaggaactatatttggtgctacaggtggagttatggaagcagcacttagaactggatatgaactttatactaaaaaaactattccaagtatagatcttactatggtaagaggtggagaaggttttagaactgctgaagtagatttaggagatattagactaaaagtaggagtagtttccggcttaaaaaatgtaaaagatgttatggaatcagtaaaggcaggtaaatgtgatttacactttatagaggttatgacttgtcctcaaggatgtataagtggtggaggacaacctaaggttatacttgattcagataaagaagaagcttataataataggaaaaagggactatataatcatgacgctaatcttacttatagaaaatcacatgaaaatccagaaataaagaaaatatatgatgagttcttagacaaaccattaggagctaagtctcatgaattattgcacactaaatatatctcaagaaaaaaggagagttaataaaatgaagaattgcctcgtagtagcagatcctaataaatgcataggatgtaggacttgtgaagcagcttgtggtattgcacattcaggaggggacttttttaatacaaatgtatccaaaattaattttaatcctcgcttaaatgtgataaaaactgctaaagtaagtgctcctgttcaatgcagacaatgcgaagatgcaccttgtggtaaagcttgtccagttaacgctatttcaaatgaaaatggttatgttagtgtagataaagatgtatgtgttggatgtaaaatctgcatgttagcttgtccttttggagctattgaattagcttctcaatataaggatggagaagttgtagaccaaaagggacttaagatgagtgaggaaggtaatcctactgtaaatggaaaaggaagagtggtagcaaataagtgtgatctttgccaggatagggatggaggacctgcttgcatagaagtttgtcctacaaaatctctcaaattagttacttatgatgacaataataatatagttgaaaaaaaagatgacgacgaacgtgaagtaggctaa